European Patent Application EP 4 631 979 A1, published October 15, 2025. Title: Novel CRISPR-Casσ enzyme and system. Applicant: CHINA AGRICULTURAL UNIVERSITY. Application US. The sequence listing filed with the application follows.

SEQUENCE LISTING (83 sequences)

SEQ ID NO: 1 - protein, 882 aa, synthetic construct
MSNYKNIKFKLVPFSQKDLINMQLNVNLHQQCYREFVEQFCVLCNIPFPGLSKDQIEQKRKQLNLSEDDEKDINYIKDLVKNKNNIGNSIYAFFTGTKKEMPSRKTDLTPLYRLLKANILPFSLLKGRENYKKSIFQTVINQTLEKFKSYFKCNESVENNFKLSLNKDSNEEQVLNESEMKDLQNLFENLSKNQSFSFFNFNKNWFSKDKIKTKLLNNETNKIKSLSSEEIDLILSYKDKLYSNEFDLISMFVEFNLQKQKAESLKSQADLNLFKNNNYSFRIGSNYENFNLTQNNKDILLEINSSMGEKITFKIIPHKKTQIWNLEKNNVKITSGENLGNYKSVDVIKMKRPADIKAKLLKTSELNIEIKNNQIYCNFIYEYKCSDHGVYFFHCSGNKKPDEKNENILKERERTFSFIDLGLFPMYSISTFKYNNKSNDGEILVKSGSGNEKLDFGSAFKIHSIQIGKNSTNLNKIKQLLEKLKDLKTYLKFSKSISSFDENSYQRQLKTGVEISELNSLSFQKISEIKSINLGFNESFNKEYFLKLIENQTFTQKELLLLNCKIKDLFKILYKEYSNIKNSRIFKFNKEDDLICDGYYWLQVIDEIINIKKSLTYFNSKPSEKGNKSKFIFLKDFNYKNNFANNYAKIAASRLKKYCLEHKVDVCVFEKNLNNFLQSKDNDKKTNKTLINWANRNLFEKIKLALEEHDICVSEVDGKHSSQLDPQTMNWGARDNLNGNGNKEKIFFERNGQIIQQNADLSASEVLAKRFFTRYEDIVHIYIDQKIKDDKTILKLVKGKVRVESYLKKTINSCYAIVDENGFLKPISKKDYNKFQELPSKPRTDIKSNEMYRHGSKWYHFQQHREFQQDLLARGRELKKIA

SEQ ID NO: 2 - protein, 935 aa, synthetic construct
MNKTDTQNNEQINKPTQLLNNKDIELTVKTVKSATVKVDNNSKKELFGLFNYFTSVASGIKDKVYNLQSDEKTAPIFNDYVKQPQRGRSAATTLFTKLDAEKTYTSQHSFPGKWRDSGIFPLYNKESEKYDLSTHGYHYSANAEIHTQLDSHDECNKECEKEYAALRDEVNNYKYEFTLQFKAENAEKFYNFVEKLTLMGWRYDATFRSFFELHMHPKLKTGETTYRATYKLPSGKSKRYSFFRDDIADEIAKNPEFWPMLESSNAISWINSNNLLSRKKDKANYSSTSLIKSQIRLYLGNNGVPFTAREHDGRIYFSFRLPAINGEKGRMVEIPCSYKKVFNGKARKSCYLGGLTIEKTDAGKHIFKYSVNNKKPQVAELNECFLRLVVRNREYFNNVVAGKITDINTDHFDFYVDLPLNVKEDPIHDLSSTEVFGKNGLRSYYSSAYPEIKNLGSQIETGKNLTCPITKTHNIMGIDLGQRNPFAYCIKDNTGKLIAQGHMDGSKNETYKKYINFGKESTSVSHLIKETRSYLHGDPEAISKELYNEVAGFCNNPVSYEEYLKYLDSKKFLINKEDLSKNAMHLLRQKDHNWIGRDWLWYISKQYKKHNENRMQDADWRQTLYWIDSLYRYIDVMKSFHNFGSFYDKNLKKKVNGTVVGFCKTVHDQINNNNDDMFKKFTNELMSVIREHKVSVVALEKMDSMLGDKSRHTFENRNYNLWPVGQLKTFMEGKLESFNVALIEIDERNTSQVCKENWSYREADDLYYVTDGESHKVHADENAANNIVDRCISRHTNMFSLHMVNPKDDYYVPTCIWDTTEESGKRVRGFLTKLYKNSDVVFTKKGDKLVKSKTSVKELKKLVGKTKEKRGQYWYRFEGKSWINEADRDTIILNAKKISRERDNGEQSTDTRSQNVTVSVLDVCETAEKKKLVLV

SEQ ID NO: 3 - protein, 900 aa, synthetic construct
MKSIKSIKSIKTKVVKNNELKLIELSTWCSSICEQLERYIFILGGKQIHDRDGVVVLDGAVERKIYCKKDKSLIAACEVVYKHFTDKSSKSRTFGSWFLGGKSEGDNTNKGRKSTKEKTEKQIAKQIADKKELTDSLQLLWDKKLLPFPIDNKGYDFINTPRAKSYKWAITKTIHAKIKSYNEQCVETKKEYDALNAEINTYKTILFSGYSEKDIDDLQKFVDICEANNHRINYKFISFLKRKDLNFDEQTGKYRKEGKWIQHKNGKEVKSKYSMKDEIVEALYKYKSLTKNDVSVLCNEHQKEDEMGKVVHYNMKRYSDLLFRKKNKKEIPSYTKISLATSKIELGLNNVKYNVEQVEDKLIWTICDQTGKDIQFVTVYTRKKEDNRTNGKKGAGFYKGKHHQLEDLKIVPVGDIGTYDISFKVNGKRPFTGTLKEPNIICRGGKVFVQMPININIDKTLNDARKKVLYAYRETYSGSVNGKKQKMIKIENSKIAESLKSLGRDAIVLGVDLGLRGLATAVVSHNGKNETVKSSQYIKGDIVEWEKYRVFNDNIREVKKYIFLTKKSYTATTEEYTEFYKECSKPEQDYLDSLKTYKDKNVKLNELKYTKNAWSVSKMFEDVSKMFETLKQDRLKYYDIFNMPYWAASLKNYMSLMKSYNYVGVDIKVSKEYMSKYQSLYNNIKEDYAKKIGSYIVQLAVAKNCDIIVLEELKSNLGSVDRKSKRDNEMSLMWNCGRIKTHVENMAKDYGMFIDEVPEYGTSQVYHKTGNYGYRDEDNREIFWYEDNKDVAYIHADENAAINIAKRFLSQHTDNSSFSVILKGDAYYLNIASNSKRMRAAALKTFGDLNKPFKINANDKNGNLYKKTRIFKSDSRWIGVNDKDLYIEHIKSLRNLRVRQ

SEQ ID NO: 4 - protein, 627 aa, synthetic construct
MPSFTKVDEDKIVLKLGNNYIPYGLSRISEDKMLWSFSSPQKKKLSIITNHRRVGKGKHFYLEGLEIADITKGDGDKTSPSGKYTISFSINGKQDVKGELKEPSFGLRNGNVYMFLPISIKQTDVFESRVEMRRLLSMAYQPTTVEDLILDDVETKQKTVKQGKKEVNTTNIAIQEAIKKHGRLLKVMGVDLGLRNFAFAIKNYDGHHDTLLRQLYSESDLNEKQRYTTLANDLSKVGNHIKFAAVFYGANDTEENTKMFDAECTDAESRTHLEWLRKAKKSGVLLKDLRKDKTWIVSIKYTELRNRLHALKFGRMKSYDYRNNLYWAATIKKFISLSASFYGVGRPSRGKKDVRELKKKHTFFSTYQDLYNNVKEDYAKKVANLVVMTAKENNVDIIVVENLTGHCGSKDYKTRAENEMSIMWNHGRIKTFIDCIANANGMLLAEVSEFETSQVYHETRNYGYRDKKMKEILWYMDSEGNVQYAHAEVNAAINIADRFLSQHTNLFSFPVCKSKKDENVYEIDIAEGKELEGQDEVKKAKKPKGGKRLNGAVVKTFGSTKIMFNGIVDKNKKGQIKTKTRVYNIDGEWGGKTQKDEYVDKIRKVVDAMSPEEKAKVKAALKKCFSS

SEQ ID NO: 5 - protein, 927 aa, synthetic construct
MTKELSGVRVIELKTDLRKDQFWDRYERCFKTYHALYNEVPCWGLDWVEQKTQNQTSRELGCERVDLTAQRKALYERTDRTISYEQFSNCLKALWLGLLNCQQGNHMYTKLFEGAIQTDQMTAEDWAVLTEYVADPKSHNSQFLFRVSNTLKHIGFFSRPPFTATLFAPERKAITKDVMSDLKGWIEMKRMTEESYAAEEVQIQQMKAEVPVRIRQSLLRFFDTCIGLNLIGHFDERVHHYLRDCIIPALQQRTIPTEHFYLKSNRKDVGQKHIDFSLDIKFYELLAEMPELWNTLETSEDDLIPKPLILKHLHLLEAIMSHRAHRKTAAYAFVGEADYHRFYYLLGGNYTKHLISATGSELPDRVIWDNDKDVLMRNGRKVERLYVKVGDRKENFNFEVYTIAMNTKGLRGHRSTLKPTSYLQDLQIWSNPEGESTYLNFVRKGTERSAICKEPVLVYRNGAFFLRLSMSVEGMRASEEHIALQYYLSAAATGSDLSKDTEKTVERFNLIQGKTYKVMSVDLGIRSPFAWAVTESTITGVANPSQILNSGEMEIADDPDYTELFYAYKNLGHLIGQVKSSSKGKGLKADSHLVDMIHTVQRFFADYKVAGQRRSQIFEQFSKDPDPLYQMDQMMKRYENNLESVKKDFSFLINILFKYVTLQFGALRNRRRSYLSQNQMADQKFDQDFKWLNILEQRKRVTRSLSYLGTDNSRIPICLEQQKLDYNGCKDNFLKQLASKIVRIAHQNDCCLIVLEDLEGYGKTLNQRDENFLTAFWSPKRVKDAIINAAQWYGIGVVTVSEAQTSQVHHESGRIGYRKGRDLFFLTPDGQIESVPSDINAAKNIGHRFFSRHTDLHQVYLKGSDEGAKRMKGCLLYQFGSLEAARTHLTGTGPTWYLDGVEWIDKTERNLRRDLLKQRVEIEKMPF

SEQ ID NO: 6 - protein, 900 aa, synthetic construct; identical to SEQ ID NO: 3

SEQ ID NO: 7 - protein, 935 aa, synthetic construct; identical to SEQ ID NO: 2

SEQ ID NO: 8 - protein, 896 aa, synthetic construct
MKKPKQNIEETDLKITTPKTATIKATNLDDKMRLFTFFNGFTTVCSKVKDDIYNFGQNEDTLPVYTDYIKASQRARMCATTLATKSECDFAKKYGEHFPLPHYNQEGMNYTTHQHTYSVNSAVHTQLDSLNECDKLTNGEYVKLKKTVDELEEKLTEEHGKEPLDFLVKFVDEQILLGWRFDGKFRLFFEVAMLPELKNGNIIYKKAYKTSGGKGRRYSFYNPSVADNISKNPTVWNLLSDVKAVDYISLSNSLLRKKPHAQYTNTTLNRAQVRPTFGNNGVPFSISVSDDDYVYIRFRLPKKDGEEKGQEISVKCSYKTSYKGKRSKTLRKSCYLGNLKIEENGKGKYICKYNINGRETTTAELNECFLRVRINNNRWFNKYLNGTLTKEDGVLKSEYFDFYFDLCLNVHQKSIHGLTNSEIFGGKGKSIRSYYSTSYPEVKNLDGQKNIKTDFGCYVDKPHNIMGIDLGQRNPFAWAVLDQNGNVKDVGHLDGAENDTYKDYLTFSNRCKDVKNLILQSRDYLYGDDEAIDETLFDSVVQFVNSNITLNKYKSYLDEKKSLINKESLEKNRLYELKKKDHGWFVRDCLWFLTKEYHRINSERKTHSDWRYTLYWVDAIHRFIDVNKSFNSLGSYYDKKQSKSINGIQKDFCRSYWNQIDNLNEDTLKKFVFELLPVIKKNNVCLIAIEELKSMLGDDDKRAEDNRLYNLWPVGQLKTFLEGKLLPYNVAVMEVSEQNTSQIVNGQWSYREGDDLYYVKNNDNNTMCKTHADENAAINIALRAYSHHTNLYSIYMINPIDDYYVPSCIWNNKDEGSKRIRGFLTKTYGTSDVVFIKKNEKLVKSDVSIKDVKRIVKNIGNEKNKKSEIWYRMNDIEWIDEGSRDIIINTIKSKVR

SEQ ID NO: 9 - protein, 887 aa, synthetic construct
MTDKSISFKQFSQILNVLYKCIVISGKGRGLTSIILGQPQCKDSLTSADWGNLETLSAKDELTPAEVKDITKDLMYRASNTLVSIGFRNRSPFKLTLTSGERYAVVENVHRSLKSWVEVDKITRENYLNEEIALSDAFNNIDETLLPTLKEFFDACMNENIIHHFDARVYAYTRDCVIPALVAGLEIKDHFYIDGRDKAKRDYSLQGYAELLKGFPKLWQGVDPEILAKLYILEAQMDHKKHRPCAAYAFIGEDSYSRVQYLLGNNYTSFSPYALGVDLDDVTCGDDAEADTQFPKNKVIQFSQGKKVTKLSLTVSRGKEDTNKYSFDVFLADKYSNGSYKPSPYFSDLSVWVSEIGMLMEFTRKGERVQAIVKEPSLIYRKGAFYVRLNMGVIQDTSPEINDLYWYLSSGAPMSMTDRSKASETPKNTERLESIKGKSYRFLGIDLGLRSPFAWAVGEASISGVINKPTIIATGDYTTARDTRYDTLFFALKNAGKVIGVTKSLANGKDASFNGLMGTITAAREYLAHYSGVATHKVAAIQAFCQDDNPLETLKGLLKSYNNDLVTLKKDPRFIGGILLRYARLLKGELVTSRKMHLREHSVESKFGQEYMWLNILEREKRVCRSLSYLGLGNDRDSVIMGNLTTPYNHCKENLLKQLAARIVSLAVENKCHVIVMESLGGSNKSMNTRGQNFLEAFWSPQKIKDTIINAAAWHGIMVAEVSESQTSQVCFETGTFGHRDRASLYFLDKNGDLQETHADMNAAKNLVERFTTRHTNLRQVNMDSLPKEGPDKTPKKSPSKKKMEKAKMDNPEDQSKRLKGFLTVKFGNVKAAQEYFASRKPEQSYSGKKDEAIYWYLDGDEWITKKEKESRVSVIEGLVGLKEVAV

SEQ ID NO: 10 - protein, 821 aa, synthetic construct
MAFQSKRRIVGNLVKEQCLKAVDGKVILTDQEKRELIKRYELHLEPYKWLLRLFLSGYEGRDDGFYEELGNTNLDKEKFFEVTAGLRDALLRQSGSSRALKSSMLGKCPPSAAVGKAAKHIQALRDAGILPFKTGLTSGEDYNVLQQAVQQLRSWVACDHRTREAYAEQQEKTSQAEEAAKKAVNEVKPEDAKSLERHERALTKLRKQERRLERMRSHAQFSLDEMDCTGYSLCMGANYLKDYCLEKEGRGLRLTLKNSTMAGSYYVSVGDGQHAGMKNPGTPAGGSPEKGRRRNILFDFAVEKCGDNYLFRYDENGKRPRAGVVKEPRFCWRRKGNSVELYLAMPINIENSMRNIFVGKQKSGKHSAFTRQWPKEVEGLDELRDAVVLGVDIGINRAAFCAALKTSRFENGLPADVQVMDTTCDALTEKGQEYRQLRKDATCLAWLIRTTRRFKADPGNKHNQIKEKDVERFDSADGAYRRYMDAIAEMPSDPLQVWEAARITGYGEWAKEIFARFNHYKHEHACCTVSLSLSDRLVWCRLIDRILSLKKCLHFGGYESKHRKGFCKSLYRLRHNARNDVRKKLARFVVDAAVDAGASVIAMEKLPSSGGKQSRDDNRIWDLMAPNTLATTVCLMAKVEGIGFVQVDPEFTSQWVFEQRVIGDREGRIVSCLDAEGVRRDYDADENAAKNIAWLALTREAEPFCMAFEKRNGVVEPKGFRFDIPEEPTREQDESNQDFKKRLEERDKLIERLQAKSDRMRAIVRRLFGDRRPWDAFADRIPEGKSKRLFRHRDGLVLNKPFKGLCGSENSEQKASARNSR

SEQ ID NO: 11 - protein, 954 aa, synthetic construct
MDTDTELSDEVELSDEVELSDEVELSDEVELTVKKVKTTTVKVDNNFKKELFELFNHFTSVASGIKDRLYDLQFDENTASIFKGYIKEAKRGHGAATTVFTKLNPKKIYSGKKSFPRDYRDRGIFPFYNKESGKYDLSTCGYHYSANAEIHTQLNSHDECNKQCEKEYAALEKERNKYKHEFTRQFKAENVEKFSNFVEKLTLMGWRYDATFRNFFELHMHPKLKTSETTYRATYKLPSGKSKRYSFSRDDIADEIAKNPEFWPMLESSNAVSWINSNNLLSRKKEKANYSSTSLIKSQIRLYLGDNGVPFTAREHDGRIYFSFRLPSINGEKGRNVEIPCSYKKVFNGKARKSCYLGGLTIENTGGSKHIFKYSVNNKKPQVAELNECFLRLVVRNHGYFNKMVNGKLTDKDGKLHADYFDFCIDLPLNVKEDPIHDLTYQEINGVKANPEKNIEKKVGLLGFYQSAYPEIKNLGSQIETGKNLTCPITKTHNIMGIDLGQRNPFAYCIKDNNGKFIAKDHMDGSKNETYKKYINFGKESTSVSHLIKETRSYLHGDPEAISKELYNEVSGLCNSPLSYEEYLKYLDSKKFLINKEDLNKNAMHLLRQKDHNWIGRDWLWYISKQYKKHNENRMQDADWRQTLYWIDSLYRYIDVMKSFHNFGSFYDKNLKKKVNGTAVGFCKTIYDQINNNNKDMFKKFTNELIPIIRKHKVSVVALEKMESMLGDKSRNTFENRNHNLWPVGQLKTFIENKLDGFNVIVVEVDERNTSQMCDGNWSYREADDLYYVKDGELREVHADENAANNIVDRCISRHTNIFSLYMTNPMDDYYVPACIWDRSENGKRGRGFLTKMYKNSDVVFTKKDDKLVKSKMSVKELKKLVDKTKEKRGQYWYLFEGKSWINAADRDTIISNAKKLFRERDGGEQSTDTRSQNVTVSVLDVCETVEKKKLVLV

SEQ ID NO: 12 - protein, 1001 aa, synthetic construct
MSTEVDVKTINLKIAKKGGVYPILEQSIKENCKSNDLLEFFMVLNRLQTYYIESNEEILVDFPKKYDELFDIVKNNDSSVTREYFDSLCDKYITEVCANGFVNNVYIAHNKNQELNWAETSNDRKIKSNKTFMFGKIKGLIRDKFGREELSDKDATKQLCEDIFNLFILNNANIELDEKYNIIKDELIQIWNERNKEFIHIKDITLLFRQWGILPTYDNITHNCELKAIIAEPVRRFKSWLECNSEANKNYDTEREKCTKYMDVMDSDLTVEFSKMVTELGNPFGANDKNIYKYFNQKFLLFFKQVVQPKFVNGEPLDESNGSYSGEIKINSAGKVENYSIAVSVIDTIKKYPTIWSDRSWGESVISTVAKIDPQYGIDDITDDMQVSPFYLFYGYFTAYNYIQQHKRNAKYTPISKDSLPSLYLGNNYIPFKIDCENVDDDRFYITIKNMNNLKLNVLYRKPKLKFAKTKEKTKRNKCYFDNLKITNTNNNFKFEYNINGDPNRSVVAYLKEPVIRYNNRKDYFYLSATISKDVETDSELTSACWSKISNDTARRVNAEQYFNDNGVNIVGIDLGMNPIIAYSVLHYKNNEFIDLNITGKIADKDKHPNLNYKRMYEKRSEIKKLKTLIKMIPDYVNSDSNIFEGDNNVFKQLDKKSKGRFRSSEYMGYYDKLNVDGKFISELEIVKKVVNTKHYKNDTEKNNDIMRVYKGNKKNIIKKEIDTHRHQIHSIKDMNRRSDESNLCYVYDMVSYIDDFKKLVTSYNKIGEDYNNPIKPLSDPMLFSKSKLYEYRQNIRDNFLKDICYQMVKIAKQYNAVLVHEHFEQRKGGIDRVNNILMALFTPNDIIKKLKCVAKREGVLVFNTNKNHTSQYVYNKNTVGYRDSNNKHNLYYIEDETTRKLGVVDSDINASKNIAARPFNKPLYAIKVKNYDDGLFLSDYNNKYVLYKKDGDKYVAIGDTYRIDKKKIKQGSVTLYLHNGYYVDGEYKNNYIENIKKLVL

SEQ ID NO: 13 - protein, 821 aa, synthetic construct
MAFQSKRRIVGNFVKEQCLKAVDGKVILTDQEKRELIKRYELHLEPHKWLLRLFLSGYEGRDDGFYEELGNTNLDKEKFFEVTAGLRDALLRQSGSSRALKSSMLGKCPPSAAVGKAAKHIQTLRDAGILPFKTGLTSGEDYNVLQQAVQQLRSWVACDHRTREAYAEQQEKTSQAEEAAKKAANEVKPEDAKSLERHERVLTKLRKQERRLERMKSHAQFSLDEMDCTGYSLCMGANYLKDYCLEKEGRGLRLTLKNSTMAGSYYVSVGDGQHAGMKNPGTPAGGSPEKGRRRNILFDFTVEKCGDNYLFRYDENGKRPRAGVVKEPRFCWRRKGNSVELYLAMPINIENSMRNIFVGKQKSGKHSAFTRQWPKEVEGLDELRDAVVLGVDIGINRAAFCAALKTSRFENGLPADVQVMDTTCDALTEKGQEYRQLRKDATCLAWLIRTTRRFKADPGNKHNQIKEKDVERFDSADGAYRRYMDAIAEMPSDPLQVWEAARITGYGEWAKEIFARFNHYKHEHACCAVSLSLSDRLVWCRLIDRILSLKKCLHFGGYESKHRKGFCKSLYRLRHNARNDVRKKLARFIVDAAVDAGASVIAMEKLPSSGGKQSKDDNRIWDLMAPNTLATTVCLMAKVEGIGFVQVDPEFTSQWVFEQRVIGDREGRIVSCLDAEGVRRDYDADENAAKNIAWLALTREAEPFCMAFEKRNGVVEPKGLRFDIPEEPTREQDESDQDFKKRLEERDKLIERLQAKADRMQAIVQRLFGDRRPWDAFADRIPEGKSKRLFRHRDGLVLNKPFKGLCGSENSGQKASARNSR

SEQ ID NO: 14 - DNA, 2649 bp, synthetic construct
  source 1..2649: mol_type = other DNA
atgagcaactacaaaaacattaagttcaagttggttccgttcagtcaaaaggatcttataaacatgcagctaaacgtgaatctccaccagcagtgttatagagagttcgtggagcagttctgcgtcctctgtaatatcccctttcctgggcttagtaaagatcaaattgagcagaagcggaaacaattaaatctgtctgaagacgacgagaaggacatcaactacatcaaggaccttgtaaaaaataagaataacatcggcaattcaatctatgcttttttcactggtacaaagaaggaaatgccaagcagaaagactgatttaacacctctttaccgcctccttaaggctaacatactgccctttagcctcctcaaagggcgagagaactataagaaaagcatattccaaactgttattaaccagacactggaaaagtttaagtcatatttcaagtgcaatgaatcagttgaaaacaacttcaaactgtctctgaacaaggactcaaatgaggagcaagtcctgaatgaaagcgaaatgaaagacctccaaaacctattcgagaatttgtctaaaaatcagtctttttccttcttcaacttcaataagaactggttctccaaggacaagatcaagacgaaactcctcaataacgagaccaacaaaattaagtcgttgtcatctgaagagatcgacctgatccttagttataaggataagttgtactccaacgaatttgatctgatttccatgttcgtggagttcaacttacagaaacagaaggcggagtccttgaaatcacaggcggacttgaacctcttcaagaacaacaactattcttttcggattggaagcaactatgaaaactttaatctaactcaaaataacaaggacatcctgctggaaatcaattcttcaatgggtgagaagattacctttaagatcattccgcataagaaaacccagatctggaatttagagaagaataatgttaagataacttcgggcgagaacctggggaattacaaatcggtggacgtcatcaagatgaagcggccagcagacattaaggcaaagctgctgaagacgtcagagctgaatatcgagatcaagaacaaccaaatctattgcaacttcatttatgagtacaagtgctccgatcatggcgtgtacttctttcactgcagtggcaacaagaagccagatgagaagaatgagaatattctaaaggagagggagaggacctttagtttcattgatctcggtctttttccgatgtattccatctccacatttaagtacaataataagagcaatgatggtgagatcctagtcaagtcgggatctgggaacgagaaactcgacttcggctctgccttcaaaattcattcaatccagattggaaagaacagcacaaatctcaacaaaattaagcaacttcttgagaagctgaaagacctgaagacctacctcaaattctctaagagcataagcagcttcgacgagaacagctaccagcgccagcttaaaacgggagtggagatcagcgagctgaacagcctgtcgttccaaaaaatatcagaaattaagtccattaatctcggcttcaatgaatccttcaataaagagtattttctaaagctgatcgaaaaccaaacattcacgcagaaggagttactactgttaaactgcaagatcaaagacctcttcaaaattctctacaaagaatattctaacatcaaaaacagtcgcatatttaaattcaataaagaagatgatctcatctgtgacgggtactactggctgcaggtcattgatgaaataatcaatattaaaaagtcgcttacttacttcaacagcaagccgtcggagaaggggaacaaaagtaagtttattttcttgaaggattttaactacaaaaataattttgcaaacaactacgcgaaaatcgctgcgtcacgtctcaaaaaatattgtttggagcacaaggttgacgtgtgtgtttttgagaagaacctcaacaactttctgcaaagcaaggacaacgataaaaagacaaataagaccttgattaattgggcgaaccgcaatctttttgagaaaattaaattggcgctggaagagcatgacatctgcgtgagtgaggttgatggtaagcattcgtcccagctggacccgcaaaccatgaactggggcgctagagataatcttaatggaaatggtaacaaagaaaagatcttttttgaaaggaacgggcagataatacaacagaacgccgacctcagtgcttctgaagtcctcgcaaaacgattcttcaccaggtacgaggacatcgtgcacatctacattgaccagaaaataaaggatgacaaaacgatccttaagttggtgaagggtaaggtgcgcgtagaatcttatctgaagaagactataaattcctgctacgccatagtagatgaaaatggcttccttaaacctatatctaagaaagactacaacaagttccaggagctgccgtccaagcctcgcacagatattaagtcgaatgagatgtacagacatggcagcaagtggtatcacttccagcaacatagggagtttcagcaggacctgttggcacggggcagagagctgaagaagatagcctga

SEQ ID NO: 15 - DNA, 2808 bp, synthetic construct
  source 1..2808: mol_type = other DNA
atgaacaagacggacacccagaacaacgagcagatcaacaagccgacgcagctgctcaacaacaaggacattgagctgacggtgaagaccgtgaagtccgcgaccgtgaaggtggacaacaacagcaagaaggagctgttcggcctgttcaactacttcaccagcgtcgcctccggcatcaaggacaaggtgtacaacctgcagtccgatgagaagaccgccccgatcttcaacgactacgtgaagcagccgcagcgcggcaggtctgctgctactactctgttcaccaagctggacgcggagaagacctacacctctcagcactccttccccggcaagtggagggattccggcatcttcccgctgtacaacaaggagtccgagaagtacgacctgtccacccacggctaccactactccgctaacgccgagatccacacccagctggacagccatgacgagtgcaacaaggagtgcgagaaggagtacgccgcccttagggacgaggtgaacaactacaagtacgagttcacgcttcagttcaaggccgagaacgccgagaagttctacaacttcgtggagaagctgacgctgatgggctggaggtacgacgctacgttcaggtctttcttcgagctgcacatgcacccaaagctcaagaccggcgagacaacgtacagggccacctacaagctgccgtccggcaagtctaagaggtacagcttcttcagggacgacatcgccgacgagattgccaagaacccagagttctggccaatgctggagtcctccaacgccatctcctggatcaactccaacaacctgctcagcaggaagaaggacaaggccaactactcctcaacctccctcatcaagtcccagattcgcctgtacctgggcaacaacggcgtgccattcaccgctagggagcacgatggcaggatttacttcagcttcaggctcccggccatcaacggcgagaagggcaggatggtcgagatcccatgcagctacaagaaggtgttcaacggcaaggccaggaagagctgctaccttggcggccttaccatcgagaagaccgacgctggcaagcatatcttcaagtactccgtgaacaacaagaagccgcaggtggccgagctgaacgagtgcttcctgaggctggttgtgaggaatagggagtacttcaacaacgtggtggccggcaagatcaccgacatcaacaccgatcacttcgacttctacgtcgatctgccgctgaacgtgaaggaggacccgatccatgatctgagcagcacggaggtgttcggcaagaatggcctgaggtcctactactcctccgcctacccagagattaagaacctgggctcccagatcgagacgggcaagaacctgacctgcccgatcaccaagacacacaacatcatgggcatcgaccttggccagcgcaacccattcgcctactgcattaaggacaacaccggcaagctcatcgcccagggccatatggacggctctaagaacgagacgtacaagaagtacatcaatttcggcaaggagtccacctccgtctcccaccttattaaggagacgaggtcctacctgcacggcgatccagaggctatctccaaggagctgtacaatgaggtcgccggcttctgcaacaacccggtttcctacgaggagtaccttaagtacctggactccaagaagttcctgatcaacaaggaggacctgtccaagaatgccatgcacctgctgaggcagaaggaccacaactggatcggcagggactggctgtggtacatcagcaagcagtacaagaagcacaacgagaacaggatgcaggacgccgactggaggcagactctgtactggatcgacagcctgtacaggtacatcgatgtgatgaagtccttccacaacttcggcagcttctacgacaagaacctgaagaagaaggtgaacggcaccgtggtgggcttctgcaagacggttcacgaccagatcaacaacaacaacgatgacatgttcaagaagttcaccaacgagctgatgagcgtgatcagggagcacaaggtgagcgtggtggcgcttgagaagatggacagcatgctgggcgacaagtcaaggcacacgttcgagaacaggaactacaacctgtggccggtgggccagctgaagacattcatggagggcaagctggagtccttcaacgtggccctgatcgagatcgatgagaggaacaccagccaggtgtgcaaggagaactggtcctacagggaggcggatgacctgtactacgtgacggacggcgagtcccacaaggtgcatgctgacgagaacgcggccaacaacatcgtggacaggtgcatttccaggcacaccaacatgttcagcctgcacatggtgaacccaaaggacgactactacgtgccgacctgcatttgggacaccacggaggagtccggcaagagggttaggggcttcctgaccaagctctacaagaactccgacgtggtcttcaccaagaagggcgacaagctggtgaagagcaagacctccgtgaaggagctgaagaagctggtgggcaagaccaaggagaagaggggccagtactggtacaggttcgagggcaagagctggatcaacgaggccgacagggacaccatcatcctgaacgccaagaagatctccagggaaagggacaacggcgagcagtccacggataccaggagccagaacgtgaccgtgtccgtgctggacgtgtgcgagacagctgagaagaagaagctggtccttgtgtga

SEQ ID NO: 16 - DNA, 2703 bp, synthetic construct
  source 1..2703: mol_type = other DNA
atgaagagcataaagagcataaaaagcatcaagacgaaggtggtgaagaacaacgagctgaagctgatagagctgagtacgtggtgcagcagcatatgcgagcagctggagaggtacatattcatcctgggggggaaacaaatacacgacagggacggcgtggtggtgctggacggcgcagtggagaggaagatctactgtaagaaagacaagagcttgatcgcggcctgcgaggtggtgtacaaacacttcacggacaagagttccaagtccaggacgtttgggtcctggttcctgggtgggaagtccgagggcgacaacaccaataagggaaggaagagtaccaaggagaagaccgagaaacaaatcgcaaagcagatcgccgacaagaaggagctgacggactccctgcaactgctgtgggacaagaagctgctgccattcccgatagacaacaagggctacgacttcataaataccccaagggccaaatcctacaagtgggcgatcacgaaaaccatccacgctaaaatcaaatcctacaacgagcaatgcgtggagaccaaaaaagagtacgacgccctgaacgccgagatcaacacctacaagaccatcctgttctccggctactccgaaaaggacatcgacgacctgcagaagttcgtggacatctgcgaggcaaacaaccacaggataaactacaaattcatatcctttctcaagaggaaagacctcaatttcgacgaacaaacagggaaatacaggaaggaaggcaagtggattcaacacaagaacggaaaggaagtcaagagcaagtacagcatgaaggacgagatagtggaggccctgtacaagtacaagtccctgacaaagaacgacgtgagcgtgctgtgcaacgagcaccaaaaagaggacgaaatgggcaaggtggtgcattacaacatgaagaggtactctgatctgctgttcagaaagaagaacaaaaaggaaatcccgagttacacgaaaatcagcctggccaccagcaagattgagttggggttgaacaatgtgaagtacaacgtggagcaggtggaggacaaactgatatggaccatatgcgaccagaccggcaaggacatccagttcgtgaccgtgtacaccaggaagaaggaggataacaggaccaatggcaagaaaggggcggggttctacaagggcaaacaccaccagctggaggacctgaaaatagtgccggtgggcgacatagggacctacgacatcagcttcaaggtgaacgggaagaggccgttcacagggaccctgaaggaaccgaacatcatatgcaggggcgggaaggtgttcgtccagatgccgatcaacatcaacatcgacaaaaccctgaacgacgcgaggaagaaggtgctgtacgcataccgggagacgtactccggctccgtgaacggcaagaagcagaagatgataaagatcgaaaactccaaaatcgccgagtccctgaaatccctggggcgggacgcgatagtcctgggcgtggatctggggctgagggggctggctacagcggtggtgagccacaacgggaaaaacgagacagtgaagagcagccaatacattaagggcgacattgtggagtgggagaagtacagggtgtttaacgacaacatcagggaggtgaagaagtacatattcctgaccaagaagtcctataccgccacgacggaggaatacaccgagttttacaaggagtgctcgaagccggagcaggactatctggactccctcaagacctataaagacaagaacgtgaaactcaacgagctgaaatacacgaagaacgcgtggtccgtgagcaagatgttcgaagacgtctccaaaatgttcgaaaccctcaagcaggacaggctgaagtactacgacatcttcaacatgccatactgggccgcctccctgaagaactacatgagcctgatgaagtcctacaactacgtcggcgtggacataaaggtgtccaaagaatacatgagcaagtaccagtccctgtacaacaacatcaaggaagattacgccaaaaaaatcggctcctacatcgtgcagctcgccgtggccaagaattgcgacatcattgtcctggaggagctgaaatccaacctcggctccgtggacaggaagagcaagagagacaacgagatgtccctgatgtggaactgcggccgcatcaagacccacgtcgagaacatggcaaaggactatgggatgttcattgacgaagtcccggagtatggcacgtcccaggtgtatcacaagaccggcaactacggctacagggatgaagacaacagggagatattttggtacgaggacaacaaggacgtggcctacatacacgccgacgagaacgcggcaatcaacatagccaaaagattcctgtcccaacataccgacaactccagcttcagcgttatcctgaagggcgacgcctactacctgaacatcgcctccaactccaaacgcatgagggccgccgcactgaaaaccttcggcgacctcaacaaaccgttcaaaatcaacgccaacgacaaaaacggaaacctgtacaagaagaccaggatcttcaagtccgactccagatggataggcgtcaacgacaaagacctctacatagaacacatcaaatccctccgcaacctccgcgtgcgccagtga

SEQ ID NO: 17 - DNA, 1884 bp, synthetic construct
  source 1..1884: mol_type = other DNA
atgccgagcttcacgaaggtggacgaggacaaaatagtgctgaagctggggaacaactacatcccgtatgggctgagcaggatttccgaggacaagatgctgtggagcttttcctccccgcaaaaaaagaagctgtctataataacgaaccacaggcgcgtcggcaagggcaaacacttttacctggaaggcttggagatcgccgacattaccaagggcgacggcgacaagacgtccccaagcggcaaatataccatctccttcagcatcaacggcaagcaggacgtgaagggcgagctgaaggagccgagcttcggcctgaggaacggcaacgtgtacatgtttctgccaatctccataaagcagaccgacgtgttcgagtccagggtggagatgaggaggttgctgtctatggcctaccagccaaccaccgtggaggatctgatcctggatgacgtggagaccaagcagaagaccgtgaagcaggggaagaaggaggtgaacaccacgaacatagcgattcaagaggcgatcaagaagcacggccgcctgctgaaggtgatgggcgtggacctggggctgaggaacttcgcgtttgccatcaagaactacgacggccaccacgacaccctgttgcggcagttgtactccgagtccgacctgaacgagaaacagaggtacactaccctggccaatgacttgtccaaggtgggcaaccacatcaagttcgccgcggtcttctacggcgccaacgacaccgaggagaacaccaagatgttcgacgccgagtgcacggacgccgagtccaggacccacctggagtggctgaggaaagccaagaagtccggtgtgctgctcaaggacctgaggaaggacaagacgtggatcgtgtcgatcaagtataccgagttgaggaataggctgcacgcactgaaattcggcaggatgaagagctacgactacaggaataacctctactgggccgcgaccattaagaagttcatctcgctctccgccagcttctacggcgtggggaggcctagccgcggcaagaaggacgtgagggagttgaagaaaaagcacaccttcttctccacgtatcaggacctgtacaacaacgtgaaggaagattacgcgaagaaggtggcgaatctggtggtgatgacggccaaagagaataacgtggacatcatcgtggtggagaacctgaccgggcactgcgggtccaaggactacaagaccagggccgagaacgagatgagtataatgtggaatcatggcaggatcaagacgttcatcgattgcatcgccaatgccaacggcatgttgttggccgaggtgtccgagttcgagacgtcccaggtgtaccacgagacgaggaactacgggtacagggacaagaagatgaaagagatcctgtggtacatggactccgaggggaacgtgcagtatgcccacgccgaggtgaacgccgccatcaatatcgccgacaggttcctgtcccagcacaccaacctgttctccttcccagtgtgcaagtccaagaaagacgagaatgtgtacgagatcgacatcgccgaggggaaagaacttgagggccaggatgaagtgaagaaggccaagaaaccgaaaggcgggaagaggctgaacggggcggtggtgaagacgtttgggagtaccaagatcatgttcaacgggatagtggacaaaaacaagaaggggcagataaagacgaagacgagggtgtacaacatagacggggagtggggggggaagacccagaaagacgagtacgtggacaaaatcaggaaggtggtggacgcgatgagcccggaggagaaagcgaaggtgaaggcggcgctgaagaagtgcttcagcagctga

SEQ ID NO: 18 - DNA, 2784 bp, synthetic construct
  source 1..2784: mol_type = other DNA
atgacgaaggagctgagcggggtgagggtgatagagctgaagaccgacctgaggaaggaccagttctgggacaggtacgagaggtgcttcaaaacgtaccacgccctgtacaacgaggtgccatgctggggcctggactgggtggagcagaaaacacaaaaccaaacctccagggaactcggctgcgagagagtggatctgaccgcccaacgcaaggcactgtatgagaggacggaccgcaccatctcttacgagcagtttagcaactgcctcaaagccctctggctggggctgctgaactgtcagcaggggaaccacatgtacaccaaactgtttgaaggcgcgatacaaaccgaccagatgaccgcggaggactgggccgtgctgaccgaatacgtcgcggacccgaagagccacaactcccagttcctgttcagggtgtccaacaccctgaagcacatcggcttcttctccaggccgccatttaccgccaccctgtttgccccagagaggaaggctattaccaaggacgtcatgtccgacctgaaaggatggattgagatgaagaggatgaccgaggagtcttacgccgcggaggaggtgcaaattcaacaaatgaaggccgaggtgccggtgcgcatcaggcagagcctgctgaggtttttcgacacctgcataggcctgaacctcatcggacacttcgacgaaagggtgcaccactacctgagggactgcataataccggcgctgcagcaaaggacgataccgaccgaacacttctacctgaaatccaaccgcaaagacgtgggccagaaacacatagacttcagcctcgacatcaaattctacgagctgctggctgaaatgccagagctgtggaacaccctggagacctccgaggacgacctcatccccaaaccgctgatcctcaaacacctgcacctgctggaagccatcatgtcccacagggcccacaggaagaccgccgcctacgccttcgtgggcgaagccgactaccacaggttctactacctgctcggcggcaactacacaaaacacctcatcagcgccaccggctccgaactgccggacagggtgatctgggacaacgacaaggacgttctgatgaggaacggcaggaaggtggagaggctgtacgtgaaagtgggcgacaggaaagagaacttcaacttcgaggtgtacacgatagcgatgaacacgaagggcctgagggggcacaggagcacgctgaagccgacgagttacttgcaagacctgcagatttggagcaacccggagggcgagagcacctatctgaacttcgtgaggaagggcacagagaggagcgcgatttgcaaagagccagtgctggtgtacaggaacggcgccttttttcttaggctgagcatgagcgtggaagggatgcgggcctccgaggagcatatcgcgctgcagtactacctttctgccgcggccacgggctctgacttgtctaaggacacggagaagaccgtggagaggttcaacttgatccaggggaagacatacaaggtgatgtccgtggatctcggcatccgctcccccttcgcctgggctgtgaccgagtcgaccatcacgggcgtggccaacccgagccagatcctgaacagcggcgagatggaaatcgcggacgacccggactataccgagctgttctacgcttacaaaaacctggggcacctgatcggccaggtcaagagcagcagcaaggggaaaggcctcaaagcggacagccacctggtggatatgattcatacggtgcaaaggttcttcgccgactacaaagtggccgggcagaggaggagtcaaatattcgagcagttcagcaaggacccggacccgttgtaccagatggaccagatgatgaagaggtacgagaacaacctggagagtgtgaagaaggattttagtttcctgataaacatcctgttcaagtacgtgaccctgcagttcggagccctgaggaaccggagaaggagctacctgtcacaaaaccagatggccgaccagaagttcgaccaagacttcaagtggctgaacatcctcgagcagaggaagcgcgtgaccaggagcctgagctacctgggcacagacaacagcaggattcctatctgcctggaacagcagaagctggactacaacggctgcaaggacaacttcctgaagcagctggcctccaagatcgtgaggatcgcccaccaaaacgactgctgcctgattgtgctggaggaccttgaggggtacgggaaaacgctcaaccagagggacgagaacttcctcacggccttctggtctccgaagagggtgaaggatgccatcatcaacgccgcccaatggtacggcattggggtggtgacggtgagcgaggcccagacgtcccaggtgcaccacgagtccggcaggatcggctatagaaaggggagggacctgtttttcctgaccccagacggccagatcgagtccgtgccgagcgacattaacgccgccaagaacattggccataggttcttttccaggcacaccgacctgcaccaggtgtacctgaagggttccgacgagggcgccaagaggatgaaaggctgccttctgtatcagttcgggagtctggaggcggcccgcacgcaccttaccggaacaggaccgacctggtacttggacggcgtggagtggatagacaagacggagaggaacctgaggagggacctgctgaagcagagggtggaaatcgagaaaatgccattctga

SEQ ID NO: 19 - DNA, 2703 bp, synthetic construct
  source 1..2703: mol_type = other DNA
atgaagagcatcaagtcgatcaagagcattaagactaaagttgtcaagaacaacgagctgaagctcatcgagctgtctacctggtgtagctcgatctgcgagcagctcgagaggtacatcttcatactgggcggcaagcagattcacgatcgcgatggcgtcgttgttctcgatggcgccgttgagcggaagatctactgcaagaaagacaagagcctgatcgccgcctgcgaggttgtctataagcactttaccgacaaatcgtccaagtctcgcacctttggcagctggttcttgggcggcaagagcgagggcgataacacaaacaagggcagaaagtccaccaaagagaagactgagaagcagatcgctaagcagatcgccgacaagaaggagctgaccgattctctgcagctcttgtgggataagaaactgctgccatttccgattgataacaagggttacgacttcatcaacacaccacgcgccaagagctacaagtgggctatcaccaagaccattcacgcgaagatcaagagctacaacgagcagtgtgtcgagacgaagaaagagtacgacgcgctgaacgccgagattaatacatacaagactattctgttcagcggttactccgagaaagacattgacgacctccagaagttcgtcgatatatgtgaggccaacaaccacaggatcaactacaagtttatcagcttcttgaagcgcaaagatttgaatttcgacgagcagacaggcaagtaccgcaaggagggcaagtggattcagcacaagaacggcaaagaagttaagtccaagtacagcatgaaagatgagatcgtcgaggcgctgtacaagtacaagagcctgactaagaacgacgtgagcgtgctctgcaacgagcatcagaaggaggacgagatgggtaaggtggtccactacaacatgaagcgctattccgacctgctgttccgcaagaagaacaagaaggaaataccaagctacacaaagatctcacttgccacgtccaagatcgagctgggcctcaacaacgtcaagtacaacgttgagcaggttgaggacaagctcatctggacaatctgcgatcaaacaggcaaagacatccagttcgtgactgtctatacaagaaagaaagaagataacaggaccaatggcaagaagggagcgggcttctataagggcaagcatcaccagctcgaagacctgaagatcgtgcctgtgggagacattggcacttacgacatcagcttcaaggtcaacggcaagcgtccgtttactggcactctgaaagagccgaacatcatttgccgcggaggcaaagtgttcgtgcagatgccaattaatatcaatatcgataagactctcaacgacgctcggaagaaggttctgtacgcctacagggagacgtacagcggctccgtcaacggtaagaaacagaagatgatcaagatcgagaacagcaagatcgccgagtcactcaagtctttgggcagagacgccattgtgcttggcgtggatttgggcttgcgcggacttgctaccgccgttgtgagccacaacggaaagaacgagactgttaagagcagccagtacatcaagggcgatattgtggagtgggagaagtacagggtgttcaatgataatatcagggaggtcaagaagtacatcttcttgaccaagaaaagctacaccgccacaacggaagaatacacagaattttacaaggagtgcagcaagcctgagcaagactatcttgatagcctcaagacgtacaaggacaagaacgttaaactgaacgaactgaagtacaccaagaacgcctggagcgtctcgaagatgtttgaagacgtttccaagatgttcgagacactcaagcaagacaggctcaagtactacgacatcttcaatatgccgtattgggcggcctcactgaagaactatatgtcgttgatgaagtcgtacaattatgttggcgtggacatcaaggtcagcaaagagtacatgtccaagtaccaatccctgtataacaacatcaaggaggactacgccaagaagatcggcagctacattgtccagctggctgtggcaaagaactgcgacatcatcgtgcttgaagagctgaagtcgaacctgggcagcgttgatcgcaagtccaagcgcgataacgaaatgagcctcatgtggaactgcggcagaatcaagactcatgtcgagaacatggccaaagattacggcatgtttatcgatgaggtgcctgagtatggtacttcgcaggtgtaccataagaccggtaactacggctatagagatgaagacaacagggaaatcttctggtacgaggataacaaagacgtcgcctacatccatgcagacgagaatgctgccatcaacatcgcgaagcgctttctgtcacagcataccgacaacagctcattctccgtgattctcaagggcgacgcttactacctgaacatcgcttccaactccaagagaatgcgcgccgccgctctcaagacctttggagatctcaacaagcctttcaagattaatgccaacgataagaacggcaacctctacaagaagacaagaatcttcaagtcagactctcgctggatcggcgtgaacgacaaggacctctacatcgagcacatcaagagcctgagaaatctcagggtgaggcagtga

SEQ ID NO: 20 - DNA, 2808 bp, synthetic construct
  source 1..2808: mol_type = other DNA
atgaacaagacggacacccagaacaacgagcagatcaacaagccgacgcagctgctcaacaacaaggacattgagctgacggtgaagaccgtgaagtccgcgaccgtgaaggtggacaacaacagcaagaaggagctgttcggcctgttcaactacttcaccagcgtcgcctccggcatcaaggacaaggtgtacaacctgcagtccgatgagaagaccgccccgatcttcaacgactacgtgaagcagccgcagcgcggcaggtctgctgctactactctgttcaccaagctggacgcggagaagacctacacctctcagcactccttccccggcaagtggagggattccggcatcttcccgctgtacaacaaggagtccgagaagtacgacctgtccacccacggctaccactactccgctaacgccgagatccacacccagctggacagccatgacgagtgcaacaaggagtgcgagaaggagtacgccgcccttagggacgaggtgaacaactacaagtacgagttcacgcttcagttcaaggccgagaacgccgagaagttctacaacttcgtggagaagctgacgctgatgggctggaggtacgacgctacgttcaggtctttcttcgagctgcacatgcacccaaagctcaagaccggcgagacaacgtacagggccacctacaagctgccgtccggcaagtctaagaggtacagcttcttcagggacgacatcgccgacgagattgccaagaacccagagttctggccaatgctggagtcctccaacgccatctcctggatcaactccaacaacctgctcagcaggaagaaggacaaggccaactactcctcaacctccctcatcaagtcccagattcgcctgtacctgggcaacaacggcgtgccattcaccgctagggagcacgatggcaggatttacttcagcttcaggctcccggccatcaacggcgagaagggcaggatggtcgagatcccatgcagctacaagaaggtgttcaacggcaaggccaggaagagctgctaccttggcggccttaccatcgagaagaccgacgctggcaagcatatcttcaagtactccgtgaacaacaagaagccgcaggtggccgagctgaacgagtgcttcctgaggctggttgtgaggaatagggagtacttcaacaacgtggtggccggcaagatcaccgacatcaacaccgatcacttcgacttctacgtcgatctgccgctgaacgtgaaggaggacccgatccatgatctgagcagcacggaggtgttcggcaagaatggcctgaggtcctactactcctccgcctacccagagattaagaacctgggctcccagatcgagaccggcaagaacctcacctgcccgatcaccaagacacacaacatcatgggcatcgaccttggccagcgcaacccattcgcctactgcattaaggacaacaccggcaagctcatcgcccagggccatatggacggctctaagaacgagacctacaagaagtacatcaatttcggcaaggagagcacctcagtctcccacctcatcaaggagaccaggagctacctgcacggcgatccagaggctatcagcaaggagctgtacaacgaggtggccggcttctgcaacaacccggtttcctacgaggagtacctcaagtacctggacagcaagaagttcctgatcaacaaggaggacctgtccaagaacgcgatgcatctcctgaggcagaaggatcacaactggatcggcagggactggctgtggtacatcagcaagcagtacaagaagcacaacgagaacaggatgcaggacgccgactggaggcagactctttactggatcgacagcctgtaccgctacatcgacgtgatgaagtccttccacaacttcggctccttctacgacaagaacctgaagaagaaggtgaacggcacggtggtgggcttctgcaagacggttcacgaccagatcaataacaacaacgacgacatgttcaagaagttcacgaatgagctgatgagcgtgatcagggagcacaaggtgagcgtggtcgcccttgagaagatggactccatgctcggcgacaagtccaggcacaccttcgagaacaggaactacaacctgtggccggttggccagctgaagacgttcatggagggcaagctggagtccttcaacgtggcgcttatcgagatcgacgagaggaacacctcccaggtttgcaaggagaactggagctacagggaggcggacgacctgtactacgtgacggacggcgagtcccacaaggtgcatgctgacgagaacgccgcgaacaacatcgtcgacaggtgcatcagcaggcacaccaacatgttcagcctgcacatggtgaacccgaaggacgactactacgtgccgacctgcatctgggacaccaccgaggagagcggcaagagggttaggggcttcctcacgaagctctacaagaactccgacgttgtcttcaccaagaagggcgacaagctggtgaagtccaagaccagcgtgaaggagctgaagaagctggttggcaagaccaaggagaagaggggccagtactggtacaggttcgagggcaagagctggatcaacgaggccgacagggacacgatcatcctgaacgcgaagaagatcagcagggagagggacaacggcgagcagtcaacggatacccggagccagaacgtgacggtgagcgttctggacgtgtgcgagaccgctgagaagaagaagctggtgctggtgtga

SEQ ID NO: 21 - DNA, 2691 bp, synthetic construct
  source 1..2691: mol_type = other DNA
atgaagaagccgaagcagaacatcgaggagacggacctgaagatcaccaccccaaagaccgcgaccatcaaggccaccaacctggacgacaagatgaggctcttcaccttcttcaacggcttcaccaccgtgtgctccaaggtgaaggacgacatctacaacttcggccagaacgaggacacactgccggtgtacaccgactacattaaggcctcccagagggccaggatgtgcgctactaccctcgctaccaagagcgagtgcgacttcgccaagaagtacggcgagcacttcccgctcccccattacaaccaggagggcatgaactacaccacccaccagcacacctactcagtgaactccgccgtgcacacacagctcgactcccttaacgagtgcgacaagctcaccaacggcgagtacgtcaagctcaagaagaccgtcgacgagctggaggagaagctgaccgaggagcacggcaaggagccacttgatttcctggtgaagttcgtggacgagcagatcctcctgggctggaggttcgacggcaagttcaggctgttcttcgaggtggcgatgctgccagagcttaagaacggcaacatcatctacaagaaggcgtacaagacctccggcggcaagggcaggaggtactctttctacaacccgtccgtggccgataacatttctaagaaccccaccgtgtggaacctgctgagcgacgttaaggcggtggactacatctccctgtctaattccctgctgaggaagaagccgcacgcccagtacaccaacacaaccctgaacagggcccaggtgaggcctacattcggcaacaacggcgtgccattctccatctccgtctccgacgacgactacgtgtacatccgcttcaggctgcccaagaaggacggcgaggagaagggccaggagatctcagtcaagtgcagctacaagacttcatacaagggcaagcgcagcaagacgctgaggaagagctgctacctgggcaacctgaagatcgaggagaatggcaagggcaagtacatttgcaagtacaacatcaacggcagggagacgaccaccgcggagcttaatgagtgcttcctgagggtgaggatcaacaacaaccgctggttcaacaagtacctgaacggcacgctgaccaaggaggacggcgttcttaagagcgagtacttcgacttctacttcgacctgtgcctgaatgtgcatcagaagtccatccacggcctgaccaactccgagattttcggcggcaagggcaagagcatcaggagctactactccacctcctacccggaggtgaagaacctggacggccagaagaacatcaagaccgacttcggctgctacgtggacaagccgcacaacatcatgggcatcgacctgggccagaggaacccattcgcctgggctgttctggaccagaacggcaatgtgaaggacgtgggccacctggacggcgctgagaacgatacatacaaggactacctgacgttctccaacaggtgcaaggacgttaagaatctgatcctgcagtccagggactacctgtacggcgacgatgaggccattgacgagaccctgttcgactccgtggtgcagttcgtgaacagcaacatcacgctgaacaagtacaagtcctacctggacgagaagaagagcctgatcaacaaggagtccctggagaagaaccgcctgtacgagctgaagaagaaggaccacggctggttcgtgagggactgcctttggttcctgaccaaggagtaccacaggatcaactccgagcgcaagacgcactccgactggaggtacaccctgtactgggtggacgccattcaccggttcattgacgtgaacaagtccttcaactccctcggcagctactacgacaagaagcagtccaagtccatcaacggcatccagaaggacttctgcaggagctactggaaccagatcgacaacctgaacgaggacaccctcaagaagttcgtgttcgagctgctgccagtgatcaagaagaacaacgtgtgcctgatcgccatcgaggagctgaagtccatgctgggcgacgacgacaagagggctgaggataacaggctgtacaacctgtggccggtgggccagcttaagacgttcctggagggcaagctgctgccgtacaacgtggctgtgatggaggtgagcgagcagaacacgagccagatcgtgaacggccagtggtcctacagggagggcgatgatctctactacgtgaagaacaacgacaacaacaccatgtgcaagacccacgcggacgagaacgcggctatcaacatcgccctgagggcctactcccaccacactaacctgtactccatctacatgatcaatccgatcgacgactactacgtcccgagctgcatctggaacaacaaggacgagggctccaagaggattaggggcttcctgaccaagacctacggcacctccgacgtggtgttcatcaagaagaatgagaagctggtgaagtccgacgtgagcatcaaggacgtgaagaggatcgtgaagaacatcggcaatgagaagaacaagaagagcgagatctggtacaggatgaacgacatcgagtggatcgacgagggcagcagggacatcatcatcaacacaatcaagagcaaggtgaggtga

SEQ ID NO: 22 - DNA, 2664 bp, synthetic construct
  source 1..2664: mol_type = other DNA
atgacggacaagagcatcagcttcaagcagttcagccagatcctcaatgtgctgtacaagtgcatcgtgatttccggcaagggccgcggccttacttccattatcctgggccagccgcagtgcaaggactcacttacctccgccgactggggcaacctggagactctttccgccaaggacgagctgacccctgctgaggttaaggatattaccaaggacctgatgtacagggccagcaacaccctggtctccatcggcttcaggaacaggtcccctttcaagctgaccctgacctccggcgagaggtacgctgttgtggagaacgtgcaccgctccctcaagtcctgggtggaggttgacaagattaccagggagaactacctcaacgaggagatcgccctgagcgatgccttcaataacatcgacgagacgctgctgccaacccttaaggagttcttcgacgcgtgcatgaatgagaacatcatccaccacttcgacgccagggtgtacgcctacacgagggattgcgtcatcccagccctggtggctggccttgagatcaaggaccacttctacatcgacggccgcgacaaggccaagagggattacagcctgcaaggttacgccgagcttctgaagggcttcccgaagctctggcagggcgttgatccggagatcctggctaagctgtacatcctggaggcccagatggaccacaagaagcacaggccatgcgccgcttacgcgttcatcggcgaggattcctacagcagggtgcagtaccttctgggcaacaactacacctccttcagcccctacgccctcggcgttgatctggatgacgtgacctgcggcgatgacgctgaggctgatacacagttccccaagaacaaggtgatccagttcagccagggcaagaaggtgaccaagctgtccctgaccgtgagcaggggcaaggaggataccaacaagtactccttcgatgtgttcctggccgacaagtacagcaacggctcctacaagccaagcccgtacttctctgacctgtccgtttgggtgagcgagatcggcatgctgatggagttcacccgcaagggcgagagggtgcaggctattgtgaaggagccatccctgatttaccgcaagggcgccttctacgtgaggcttaatatgggcgtgattcaggacacctccccggagatcaacgacctgtactggtacttgtcctccggcgccccaatgtccatgaccgataggtccaaggcttccgagaccccgaagaacaccgagaggctggagtcaattaagggcaagagctaccgcttcctgggcatcgacctgggccttaggtccccattcgcctgggctgttggcgaggcttctatctccggcgtcatcaacaagccgacgatcattgccaccggcgactacaccaccgccagggatactaggtacgacacgctcttcttcgccctcaagaatgcgggcaaggtgattggcgtgaccaagtccctcgccaacggcaaggacgcttctttcaatggcctgatgggcaccatcaccgccgctagggagtaccttgcgcactactccggcgtcgctacccataaggtggccgctatccaggccttctgccaggatgacaacccgctggagacccttaagggcctgctcaagtcctacaacaacgacctcgtcaccctcaagaaggaccctaggttcatcggcggcatcctgctcaggtacgccaggcttctgaagggcgagcttgtgacctccaggaagatgcacctgcgggagcactccgtggagtctaagttcggccaggagtacatgtggctgaatattctggagagggagaagagggtgtgcaggagcctgtcctacctgggccttggcaacgacagggacagcgttatcatgggcaacctgaccacgccgtacaaccactgcaaggagaacctgcttaagcagctggccgcgaggattgtgtcactggctgtggagaataagtgccacgttatcgtgatggagtccctgggcggctccaacaagtccatgaataccaggggccagaacttcctcgaggccttctggtccccacagaagatcaaggacaccatcatcaacgccgccgcctggcatggcatcatggttgctgaggtgagcgagagccagacctcccaggtttgcttcgagaccggcaccttcggccacagggatagggcttctctgtacttcctggacaagaacggcgacctccaggagacgcatgccgatatgaacgccgccaagaacctcgtggagaggttcaccaccaggcacaccaacctgaggcaggtgaatatggactccctccccaaggagggcccggataagacaccaaagaagtccccgtccaagaagaagatggagaaggcgaagatggacaacccagaggaccagtccaagaggctcaagggcttcctgaccgtgaagttcggcaatgtgaaggccgcccaggagtacttcgcctctaggaagccggagcagagctacagcggcaagaaggacgaggccatctactggtacttggacggcgacgagtggatcaccaagaaggagaaggagtccagggtcagcgtgattgagggcctggtgggccttaaggaggtggctgtttga

SEQ ID NO: 23 - DNA, 2466 bp, synthetic construct
  source 1..2466: mol_type = other DNA
atggcgttccagagcaagaggaggattgtgggcaacctggtgaaggagcagtgcctcaaggccgtggatggcaaggtgatcctgaccgaccaggagaagagggagctgatcaagaggtacgagctgcacctggagccgtacaagtggctgctgaggctgttcctgtccggctacgagggcagggatgacggcttctacgaggagctgggcaacacgaacctggacaaggagaagttcttcgaggtcaccgcgggcctcagggatgctcttcttaggcagtctggctcctccagggcgcttaagtcctccatgctgggcaagtgcccgccatcagctgctgttggcaaggctgctaagcacatccaggctctgcgcgacgctggcattcttccattcaagacgggcctcacctccggcgaggattacaacgtgcttcagcaggccgtccagcagctgaggtcatgggttgcttgcgatcacaggaccagggaggcgtacgctgagcagcaggagaagacatcccaggccgaggaggctgctaagaaggctgtgaacgaggtgaagccagaggacgccaagagcctggagaggcatgagagggctctgacgaagctgaggaagcaggagaggaggctggagaggatgaggagccacgctcagttcagcctggacgagatggactgcacgggctacagcctgtgcatgggcgctaactacctgaaggactactgcctggagaaggagggcaggggccttaggcttaccctgaagaatagcactatggccggcagctactacgtttccgtgggcgatggccagcacgctggcatgaagaacccaggtactccggcgggcggctctccagagaagggcaggaggaggaacatcctgttcgacttcgcggttgagaagtgcggcgacaactaccttttcaggtacgacgagaacggcaagcgcccgagggctggcgttgttaaggagccaaggttctgctggaggcggaagggcaactccgtggagctttacctggccatgccgatcaacatcgagaacagcatgaggaacatcttcgtcggcaagcagaagagcggcaagcactccgctttcacccggcagtggccaaaggaggtggagggccttgacgagctgagggatgctgtggtgctgggcgttgacatcggcatcaacagggcggctttctgcgcggctctgaagacttcccgcttcgagaacggcctgccggctgatgttcaggttatggataccacctgcgatgctctgaccgagaagggccaggagtacaggcagctgaggaaggacgccacctgccttgcttggctgatcaggacaaccaggaggttcaaggccgacccaggtaacaagcacaaccagatcaaggagaaggacgtggagaggttcgacagcgccgacggcgcttacaggaggtacatggacgccatcgcggagatgccgtccgatccacttcaggtgtgggaggctgccaggatcaccggctacggcgagtgggctaaggagattttcgccaggttcaatcactacaagcacgagcatgcctgctgcaccgtctccctttccctgtctgaccgcctggtgtggtgcaggcttatcgataggatcttgtctctcaagaagtgccttcacttcggcggctacgagtccaagcacaggaagggcttctgcaagtccctctacaggcttaggcacaatgccaggaacgacgtcaggaagaagctggccaggttcgtggtggacgccgctgttgatgcgggcgcttctgttatcgcgatggaaaagctcccgtcctccggcggcaagcagtctagggatgacaaccggatctgggacctgatggccccaaacaccctggctaccaccgtgtgcctcatggctaaggttgagggcatcggcttcgtgcaggtggacccagagttcacctcccagtgggtgttcgagcagagggtgattggcgatagggagggcaggattgtgtcctgcctggacgctgagggcgtgaggagggattacgacgctgacgagaacgccgcgaagaacatcgcctggctggctcttactagggaggcggagccattctgcatggccttcgagaagcggaatggcgtggtggagccgaagggcttcaggttcgacattccggaggagccgaccagggagcaggatgagtcaaaccaggacttcaagaagaggctggaggagagggacaagctgatcgagaggctgcaggcgaagagcgataggatgagggcgatcgtgaggaggctcttcggcgataggaggccgtgggatgctttcgctgacaggattcctgagggcaagtccaagaggctgttccggcacagggatggcctggttctgaacaagccgttcaagggcctgtgcggctccgagaatagcgagcagaaggcctccgccaggaactctaggtga

SEQ ID NO: 24 - DNA, 2865 bp, synthetic construct
  source 1..2865: mol_type = other DNA
atggacacggacacggagctgagcgacgaggttgagctgagcgatgaggtggagctgagcgacgaggtggagctttccgacgaggtggagctgacggtgaagaaggtgaagacgacgacggtgaaggtggacaacaatttcaagaaggagctgttcgagctgttcaatcacttcaccagcgtggcgagcggcatcaaggacaggctttacgacctgcagttcgatgagaacactgcctccatcttcaagggctacatcaaggaggccaagaggggccacggcgctgctactactgtgttcactaagctgaacccgaagaagatctactccggcaagaagtccttcccaagggattacagggaccggggcatcttcccgttctacaacaaggagtctggcaagtacgacctgtccacctgcggctaccactacagcgctaacgccgagattcacacccagctcaacagccacgacgagtgcaacaagcagtgcgagaaggagtacgcggcgctggagaaggagaggaacaagtacaagcatgagttcacgaggcagttcaaggccgagaacgtggagaagttcagcaacttcgtggagaagctgacactgatgggctggaggtacgatgcgaccttcaggaacttcttcgagctgcacatgcacccaaagctcaagacgtccgagaccacctacagggccacctacaagctgccgtccggcaagtctaagcggtactccttctccagggacgatattgccgacgagatcgccaagaaccccgagttctggccaatgctggagtcctccaacgccgtttcctggatcaactccaacaatctgctctccaggaagaaggagaaggccaattactccagcaccagcctgatcaagtcccagattaggctgtacctgggcgacaacggcgtgccattcaccgctagggagcacgatggcaggatctacttcagcttcaggctcccgtccatcaacggcgagaagggcaggaacgtcgagatcccatgctcctacaagaaggtcttcaatggcaaggccaggaagtcctgctacctgggcggccttaccatcgagaacaccggcggctcaaagcacattttcaagtactccgtgaacaacaagaagccgcaggtggcggagctgaacgagtgcttcctgaggctggtcgtgaggaatcatggctacttcaacaagatggtgaacggcaagctcacggataaggacggcaagctgcacgccgactacttcgatttctgcatcgacctgccgcttaacgtgaaggaggacccgatccacgacctgacctaccaggagattaacggcgtgaaggccaacccggagaagaacatcgagaagaaggtgggcctgctgggcttctaccagtccgcttacccagagatcaagaacctcggctcccagatcgagaccggcaagaacctgacctgcccgatcaccaagacccacaacatcatgggcatcgacctcggccagcgcaacccattcgcttactgcatcaaggacaacaacggcaagttcatcgcgaaggaccacatggacggctccaagaacgagacatacaagaagtacatcaatttcggcaaggagagcacctcagtctcccacctgatcaaggagaccaggtcctacctgcatggcgatccggaggctatctccaaggagctgtacaacgaggtcagcggcctgtgcaactctccgcttagctacgaggagtaccttaagtacctggacagcaagaagttcctgatcaacaaggaggacctgaacaagaacgccatgcacctgctgaggcagaaggaccacaactggatcggcagggactggctgtggtacatcagcaagcagtacaagaagcacaacgagaacaggatgcaggacgccgactggaggcagactctgtactggatcgacagcctgtacaggtacatcgatgtgatgaagtccttccacaacttcggcagcttctacgacaagaacctgaagaagaaggtgaacggcaccgccgtgggcttctgcaagactatctacgaccagatcaacaacaacaacaaggacatgttcaagaagttcaccaatgagctgatcccgatcatccgcaagcacaaggtgtccgtggtggcccttgagaagatggagtccatgctgggcgacaagtccaggaacacattcgagaacaggaaccacaacctgtggccagtcggccagctgaagaccttcatcgagaacaagctggatggcttcaacgtgatcgtggtggaggtggacgagaggaacacgagccagatgtgcgacggcaactggtcctacagggaggctgacgacctctactacgtcaaggacggcgagctgagggaggttcacgctgatgagaatgcggccaacaacatcgtcgacaggtgcatctccaggcataccaacatcttcagcctgtacatgaccaacccgatggacgactactacgtgccggcgtgcatctgggacaggtcagagaatggcaagaggggcaggggcttcctgaccaagatgtacaagaacagcgacgtggtgttcaccaagaaggacgacaagctggtgaagtccaagatgtccgtgaaggagctgaagaagctggtggacaagaccaaggagaagaggggccagtactggtacttgttcgagggcaagagctggatcaacgccgccgatagggataccattatctccaacgcgaagaagctcttcagggagagggatggcggcgagcagtcaactgatacccgctctcagaacgtgacggtgtccgtgctggacgtgtgcgagactgtggagaagaagaagctggtcctggtgtga

SEQ ID NO: 25 - DNA, 3006 bp, synthetic construct
  source 1..3006: mol_type = other DNA
atgagcacggaggtggacgtgaagacgatcaacctgaagatcgcgaagaagggcggcgtgtacccgattctggagcagtcaattaaggagaactgcaagagcaacgacctgctggagttcttcatggtgctgaacaggctgcagacctactacatcgagagcaacgaggagattctggtggacttccccaagaagtacgacgagctgttcgacatcgtgaagaacaacgactcctccgtgaccagggaatacttcgactccctctgcgacaagtacatcacagaggtgtgcgccaatggcttcgtcaacaacgtgtacattgcccacaacaagaaccaggagctgaactgggctgagacgagcaacgaccgcaagatcaagagcaacaagaccttcatgttcggcaagatcaagggcctgatccgcgacaagttcggcagggaggagctgtcagacaaggacgctacgaagcagctgtgcgaggacatcttcaacctcttcatcctgaacaacgccaacatcgagctggacgagaagtacaacatcatcaaggacgagctgatccagatctggaacgagaggaacaaggagttcatccacatcaaggacatcaccctgctgttcaggcagtggggcatcctgcctacctacgacaacatcacccacaactgcgagctgaaggccatcatcgccgagccagtgaggaggttcaagtcctggctggagtgcaactctgaggcgaacaagaactacgacaccgagagggagaagtgcaccaagtacatggacgtgatggactccgacctgaccgtggagttcagcaagatggtgacggagctgggcaacccattcggcgctaacgacaagaacatctacaagtacttcaaccagaagttcctcctgttcttcaagcaggttgtgcagcccaagttcgttaacggcgagccgctggacgagtctaatggctcttactccggcgagatcaagatcaactccgcgggcaaggtggagaactactccatcgccgtgtccgtgattgacaccatcaagaagtacccgacgatctggtccgaccgctcctggggcgagtctgttatctccaccgtggccaagattgatccgcagtacggcatcgacgacatcaccgacgatatgcaggtgtccccgttctacctcttctacggctacttcaccgcctacaactacatccagcagcacaagaggaacgccaagtacaccccgatctccaaggactccctgccatccctgtacctcggcaacaactacatcccattcaagatcgactgcgagaacgtcgacgacgaccggttctacatcaccatcaagaacatgaacaacctgaagctgaacgtcctctaccgcaagcccaagctgaagttcgccaagaccaaggagaagaccaagaggaacaagtgctacttcgacaacctcaagatcaccaacaccaacaacaacttcaagttcgagtacaacatcaacggcgacccaaacaggtccgtggtggcttacctgaaggagccagtgatccgctacaacaacaggaaggactacttctacctgagcgccacaatcagcaaggacgtggagaccgactccgagctgacctctgcttgctggtcgaagatctccaacgacaccgcccgcagggtcaacgctgagcagtacttcaacgacaacggcgtgaacatcgtgggcattgacctgggcatgaacccgatcatcgcctactctgttctgcactacaagaacaacgagttcattgacctgaacattaccggcaagatcgccgacaaggataagcaccccaatctgaactacaagaggatgtacgagaagaggtccgagatcaagaagctcaagaccctgatcaagatgatcccggactacgtgaacagcgacagcaacatcttcgagggcgacaataacgtgttcaagcagctggacaagaagagcaagggcaggttcaggtcctccgagtacatgggctactacgacaagctgaacgtggacggcaagttcatctccgagctggagatcgtgaagaaggtggtgaacacaaagcactacaagaatgacaccgagaagaacaacgatattatgagggtgtacaagggcaataagaagaacatcatcaagaaggagatcgacacccacaggcaccagatccactccatcaaggacatgaacaggaggtccgacgagagcaacctgtgctacgtgtacgacatggtgagctacatcgacgacttcaagaagctggtgacctcctacaacaagatcggcgaggactacaacaacccgatcaagccgctgagcgacccgatgcttttctccaagtccaagctgtacgagtacaggcagaacatcagggacaatttcctgaaggacatctgctaccagatggtgaagatcgccaagcagtacaatgccgtgctggtgcacgagcacttcgagcagaggaagggcggcattgacagggtgaacaacatcctgatggccctgttcacgccgaacgacatcatcaagaagctgaagtgcgtggccaagagggagggcgttctggttttcaacaccaacaagaaccatacctcccagtacgtgtacaacaagaacaccgtcggctaccgcgacagcaacaacaagcacaacctgtactacatcgaggacgagaccaccaggaagctcggcgttgtggactccgacatcaacgcctccaagaacatcgccgcccgcccattcaacaagccactctacgccatcaaggtgaagaactacgatgacggcctgttcctgtcagactacaacaataagtacgttctgtacaagaaggacggcgacaagtacgtggccatcggcgatacatacaggatcgacaagaagaagatcaagcagggctccgtgaccctgtacctgcataacggctactacgtggatggcgagtacaagaacaattacatcgagaatatcaagaagctggtcctgtga

SEQ ID NO: 26 - DNA, 2466 bp, synthetic construct
  source 1..2466: mol_type = other DNA
atggcgttccagagcaagaggaggattgtgggcaacttcgtgaaggagcagtgcctgaaggccgtggatggcaaggtgatcctgacggaccaggagaagagggagctgattaagaggtacgagctgcacctggagccgcataagtggctgctgaggctgttcctgtccggctacgagggcagggatgacggcttctacgaggagctgggcaacacgaacctggacaaggagaagttcttcgaggtcaccgcgggcctgagggatgctcttcttaggcagtctggcagcagcagggcgcttaagtcctccatgctgggcaagtgcccgccatcagctgctgttggcaaggctgctaagcacatccagaccctgagggacgccggcattctcccattcaagacgggcctgacctccggcgaggattacaacgtgctgcagcaggccgtgcagcagcttaggtcatgggtggcttgcgaccacaggacgagggaggcttacgctgagcagcaggagaagacaagccaggccgaggaggctgctaagaaggctgctaacgaggtgaagccggaggatgcgaagtctctggagaggcacgagagggtgctgacgaagctgaggaagcaggagaggaggctggagaggatgaagagccacgcgcagttcagcctggacgagatggactgcacgggctactccctgtgcatgggcgctaattacctgaaggactactgcctggagaaggagggcaggggccttaggcttaccctgaagaatagcacgatggctggcagctactacgtttccgtgggcgacggccagcacgctggcatgaagaatccgggcaccccagctggcggctctccagagaagggcaggaggaggaatatcctgttcgacttcaccgtggagaagtgcggcgacaattacctgttcaggtacgacgagaacggcaagaggccgagggctggcgttgttaaggagccaaggttctgctggaggcggaagggcaacagcgtggagctttacctggcgatgccgatcaacatcgagaacagcatgaggaacatcttcgtgggcaagcagaagtccggcaagcactccgctttcacccggcagtggccaaaggaggtcgagggccttgacgagcttagggacgctgtggtgctgggcgttgacatcggcatcaacagggcggctttctgcgccgctctgaagacttccaggttcgagaatggcctgccggccgatgtgcaggttatggataccacctgcgatgcgctgaccgagaagggccaggagtacaggcagctgaggaaggacgccacctgccttgcttggctgatcaggacgaccaggaggttcaaggctgacccaggtaacaagcacaaccagatcaaggagaaggacgtggagaggttcgacagcgccgacggcgcttacaggaggtacatggacgccatcgcggagatgccgagcgatccacttcaggtctgggaggctgccaggatcaccggctacggcgagtgggctaaggagattttcgccaggttcaaccactacaagcatgagcacgcctgctgcgccgtgtctctttctctttccgacaggctggtgtggtgcaggctcatcgacaggatcttgtctctgaagaagtgcctccacttcggcggctacgagtccaagcacaggaagggcttctgcaagtccctgtacaggctgaggcacaacgccaggaacgacgtgaggaagaagctggccaggttcatcgtggatgccgccgttgacgcgggcgcttctgttattgcgatggagaagctgccgtcctctggcggcaagcagtcaaaggacgacaacaggatctgggacctgatggccccgaacaccctggctactactgtgtgcctgatggccaaggtggagggcatcggcttcgtccaggtcgatccagagttcacctcccagtgggtgttcgagcagagggtgattggcgatagggagggcaggatcgtgagctgcctggatgctgagggcgtgaggagggattacgacgctgacgagaacgccgcgaagaacatcgcctggctggctcttaccagggaggctgagccattctgcatggcgttcgagaagaggaacggcgtggtggagccgaagggccttaggttcgacatcccggaggagcctaccagggagcaggatgagtcggaccaggacttcaagaagaggctggaggagagggacaagctgatcgagaggctgcaggcgaaggcggataggatgcaggctatcgttcagaggcttttcggcgacaggaggccgtgggatgctttcgctgacaggattcctgagggcaagagcaagaggctgttcaggcacagggacggcctggttctgaacaagccgttcaagggcctgtgcggctccgagaatagcggccagaaggcttctgctaggaacagccgctga

SEQ ID NO: 27 - RNA, 36 nt, synthetic construct
  source 1..36: mol_type = other RNA
agtgcaatagttacagaatagtaattatattcgcac

SEQ ID NO: 28 - RNA, 34 nt, synthetic construct
  source 1..34: mol_type = other RNA
tgttggtatctagtaaaatctagagccgttgaca

SEQ ID NO: 29 - RNA, 30 nt, synthetic construct
  source 1..30: mol_type = other RNA
gtgtcaacgcatcctctatagttgaggaag

SEQ ID NO: 30 - RNA, 36 nt, synthetic construct
  source 1..36: mol_type = other RNA
gtgttgtcctcattataatatgatggacagagacac

SEQ ID NO: 31 - RNA, 36 nt, synthetic construct
  source 1..36: mol_type = other RNA
ctaactgtgtgagcttctaaccgaagctaatgacac

SEQ ID NO: 32 - RNA, 36 nt, synthetic construct
  source 1..36: mol_type = other RNA
gtgtcaacgcatcctctatagttgaggaagcaacac

SEQ ID NO: 33 - RNA, 37 nt, synthetic construct
  source 1..37: mol_type = other RNA
gtgtcaacggctctagattttactagataccaacaca

SEQ ID NO: 34 - RNA, 36 nt, synthetic construct
  source 1..36: mol_type = other RNA
gtgttagtatcttgtagaatcaggagctattgacac

SEQ ID NO: 35 - RNA, 36 nt, synthetic construct
  source 1..36: mol_type = other RNA
gtgtcaatgatccattttatggatccacactgagat

SEQ ID NO: 36 - RNA, 36 nt, synthetic construct
  source 1..36: mol_type = other RNA
gtgtcattagccaccccattcagaggaggcctacac

SEQ ID NO: 37 - RNA, 36 nt, synthetic construct
  source 1..36: mol_type = other RNA
gtgttggtatctagtaaaatctagagccgttgacac

SEQ ID NO: 38 - RNA, 36 nt, synthetic construct
  source 1..36: mol_type = other RNA
atagtcgagggtgtaataatatgcacctaatgcgac

SEQ ID NO: 39 - RNA, 36 nt, synthetic construct
  source 1..36: mol_type = other RNA
gtgtaggcctcctctgaatggggtggctaatgacac

SEQ ID NO: 40 - DNA, 36 bp, synthetic construct
  source 1..36: mol_type = other DNA
agtgcaatagttacagaatagtaattatattcgcac

SEQ ID NO: 41 - DNA, 34 bp, synthetic construct
  source 1..34: mol_type = other DNA
tgttggtatctagtaaaatctagagccgttgaca

SEQ ID NO: 42 - DNA, 30 bp, synthetic construct
  source 1..30: mol_type = other DNA
gtgtcaacgcatcctctatagttgaggaag

SEQ ID NO: 43 - DNA, 36 bp, synthetic construct
  source 1..36: mol_type = other DNA
gtgttgtcctcattataatatgatggacagagacac

SEQ ID NO: 44 - DNA, 36 bp, synthetic construct
  source 1..36: mol_type = other DNA
ctaactgtgtgagcttctaaccgaagctaatgacac

SEQ ID NO: 45 - DNA, 36 bp, synthetic construct
  source 1..36: mol_type = other DNA
gtgtcaacgcatcctctatagttgaggaagcaacac

SEQ ID NO: 46 - DNA, 37 bp, synthetic construct
  source 1..37: mol_type = other DNA
gtgtcaacggctctagattttactagataccaacaca

SEQ ID NO: 47 - DNA, 36 bp, synthetic construct
  source 1..36: mol_type = other DNA
gtgttagtatcttgtagaatcaggagctattgacac

SEQ ID NO: 48 - DNA, 36 bp, synthetic construct
  source 1..36: mol_type = other DNA
gtgtcaatgatccattttatggatccacactgagat

SEQ ID NO: 49 - DNA, 36 bp, synthetic construct
  source 1..36: mol_type = other DNA
gtgtcattagccaccccattcagaggaggcctacac

SEQ ID NO: 50 - DNA, 36 bp, synthetic construct
  source 1..36: mol_type = other DNA
gtgttggtatctagtaaaatctagagccgttgacac

SEQ ID NO: 51 - DNA, 36 bp, synthetic construct
  source 1..36: mol_type = other DNA
atagtcgagggtgtaataatatgcacctaatgcgac

SEQ ID NO: 52 - DNA, 36 bp, synthetic construct
  source 1..36: mol_type = other DNA
gtgtaggcctcctctgaatggggtggctaatgacac

SEQ ID NO: 53 - protein, 11 aa, synthetic construct
SRADPKKKRKV

SEQ ID NO: 54 - protein, 925 aa, synthetic construct
MGPKKKRKVMDYKDHDGDYKDHDIDYKDDDDKMSNYKNIKFKLVPFSQKDLINMQLNVNLHQQCYREFVEQFCVLCNIPFPGLSKDQIEQKRKQLNLSEDDEKDINYIKDLVKNKNNIGNSIYAFFTGTKKEMPSRKTDLTPLYRLLKANILPFSLLKGRENYKKSIFQTVINQTLEKFKSYFKCNESVENNFKLSLNKDSNEEQVLNESEMKDLQNLFENLSKNQSFSFFNFNKNWFSKDKIKTKLLNNETNKIKSLSSEEIDLILSYKDKLYSNEFDLISMFVEFNLQKQKAESLKSQADLNLFKNNNYSFRIGSNYENFNLTQNNKDILLEINSSMGEKITFKIIPHKKTQIWNLEKNNVKITSGENLGNYKSVDVIKMKRPADIKAKLLKTSELNIEIKNNQIYCNFIYEYKCSDHGVYFFHCSGNKKPDEKNENILKERERTFSFIDLGLFPMYSISTFKYNNKSNDGEILVKSGSGNEKLDFGSAFKIHSIQIGKNSTNLNKIKQLLEKLKDLKTYLKFSKSISSFDENSYQRQLKTGVEISELNSLSFQKISEIKSINLGFNESFNKEYFLKLIENQTFTQKELLLLNCKIKDLFKILYKEYSNIKNSRIFKFNKEDDLICDGYYWLQVIDEIINIKKSLTYFNSKPSEKGNKSKFIFLKDFNYKNNFANNYAKIAASRLKKYCLEHKVDVCVFEKNLNNFLQSKDNDKKTNKTLINWANRNLFEKIKLALEEHDICVSEVDGKHSSQLDPQTMNWGARDNLNGNGNKEKIFFERNGQIIQQNADLSASEVLAKRFFTRYEDIVHIYIDQKIKDDKTILKLVKGKVRVESYLKKTINSCYAIVDENGFLKPISKKDYNKFQELPSKPRTDIKSNEMYRHGSKWYHFQQHREFQQDLLARGRELKKIASRADPKKKRKV

SEQ ID NO: 55 - protein, 978 aa, synthetic construct
MGPKKKRKVMDYKDHDGDYKDHDIDYKDDDDKMNKTDTQNNEQINKPTQLLNNKDIELTVKTVKSATVKVDNNSKKELFGLFNYFTSVASGIKDKVYNLQSDEKTAPIFNDYVKQPQRGRSAATTLFTKLDAEKTYTSQHSFPGKWRDSGIFPLYNKESEKYDLSTHGYHYSANAEIHTQLDSHDECNKECEKEYAALRDEVNNYKYEFTLQFKAENAEKFYNFVEKLTLMGWRYDATFRSFFELHMHPKLKTGETTYRATYKLPSGKSKRYSFFRDDIADEIAKNPEFWPMLESSNAISWINSNNLLSRKKDKANYSSTSLIKSQIRLYLGNNGVPFTAREHDGRIYFSFRLPAINGEKGRMVEIPCSYKKVFNGKARKSCYLGGLTIEKTDAGKHIFKYSVNNKKPQVAELNECFLRLVVRNREYFNNVVAGKITDINTDHFDFYVDLPLNVKEDPIHDLSSTEVFGKNGLRSYYSSAYPEIKNLGSQIETGKNLTCPITKTHNIMGIDLGQRNPFAYCIKDNTGKLIAQGHMDGSKNETYKKYINFGKESTSVSHLIKETRSYLHGDPEAISKELYNEVAGFCNNPVSYEEYLKYLDSKKFLINKEDLSKNAMHLLRQKDHNWIGRDWLWYISKQYKKHNENRMQDADWRQTLYWIDSLYRYIDVMKSFHNFGSFYDKNLKKKVNGTVVGFCKTVHDQINNNNDDMFKKFTNELMSVIREHKVSVVALEKMDSMLGDKSRHTFENRNYNLWPVGQLKTFMEGKLESFNVALIEIDERNTSQVCKENWSYREADDLYYVTDGESHKVHADENAANNIVDRCISRHTNMFSLHMVNPKDDYYVPTCIWDTTEESGKRVRGFLTKLYKNSDVVFTKKGDKLVKSKTSVKELKKLVGKTKEKRGQYWYRFEGKSWINEADRDTIILNAKKISRERDNGEQSTDTRSQNVTVSVLDVCETAEKKKLVLVSRADPKKKRKV

SEQ ID NO: 56 - protein, 943 aa, synthetic construct
MGPKKKRKVMDYKDHDGDYKDHDIDYKDDDDKMKSIKSIKSIKTKVVKNNELKLIELSTWCSSICEQLERYIFILGGKQIHDRDGVVVLDGAVERKIYCKKDKSLIAACEVVYKHFTDKSSKSRTFGSWFLGGKSEGDNTNKGRKSTKEKTEKQIAKQIADKKELTDSLQLLWDKKLLPFPIDNKGYDFINTPRAKSYKWAITKTIHAKIKSYNEQCVETKKEYDALNAEINTYKTILFSGYSEKDIDDLQKFVDICEANNHRINYKFISFLKRKDLNFDEQTGKYRKEGKWIQHKNGKEVKSKYSMKDEIVEALYKYKSLTKNDVSVLCNEHQKEDEMGKVVHYNMKRYSDLLFRKKNKKEIPSYTKISLATSKIELGLNNVKYNVEQVEDKLIWTICDQTGKDIQFVTVYTRKKEDNRTNGKKGAGFYKGKHHQLEDLKIVPVGDIGTYDISFKVNGKRPFTGTLKEPNIICRGGKVFVQMPININIDKTLNDARKKVLYAYRETYSGSVNGKKQKMIKIENSKIAESLKSLGRDAIVLGVDLGLRGLATAVVSHNGKNETVKSSQYIKGDIVEWEKYRVFNDNIREVKKYIFLTKKSYTATTEEYTEFYKECSKPEQDYLDSLKTYKDKNVKLNELKYTKNAWSVSKMFEDVSKMFETLKQDRLKYYDIFNMPYWAASLKNYMSLMKSYNYVGVDIKVSKEYMSKYQSLYNNIKEDYAKKIGSYIVQLAVAKNCDIIVLEELKSNLGSVDRKSKRDNEMSLMWNCGRIKTHVENMAKDYGMFIDEVPEYGTSQVYHKTGNYGYRDEDNREIFWYEDNKDVAYIHADENAAINIAKRFLSQHTDNSSFSVILKGDAYYLNIASNSKRMRAAALKTFGDLNKPFKINANDKNGNLYKKTRIFKSDSRWIGVNDKDLYIEHIKSLRNLRVRQSRADPKKKRKV

SEQ ID NO: 57 - protein, 670 aa, synthetic construct
MGPKKKRKVMDYKDHDGDYKDHDIDYKDDDDKMPSFTKVDEDKIVLKLGNNYIPYGLSRISEDKMLWSFSSPQKKKLSIITNHRRVGKGKHFYLEGLEIADITKGDGDKTSPSGKYTISFSINGKQDVKGELKEPSFGLRNGNVYMFLPISIKQTDVFESRVEMRRLLSMAYQPTTVEDLILDDVETKQKTVKQGKKEVNTTNIAIQEAIKKHGRLLKVMGVDLGLRNFAFAIKNYDGHHDTLLRQLYSESDLNEKQRYTTLANDLSKVGNHIKFAAVFYGANDTEENTKMFDAECTDAESRTHLEWLRKAKKSGVLLKDLRKDKTWIVSIKYTELRNRLHALKFGRMKSYDYRNNLYWAATIKKFISLSASFYGVGRPSRGKKDVRELKKKHTFFSTYQDLYNNVKEDYAKKVANLVVMTAKENNVDIIVVENLTGHCGSKDYKTRAENEMSIMWNHGRIKTFIDCIANANGMLLAEVSEFETSQVYHETRNYGYRDKKMKEILWYMDSEGNVQYAHAEVNAAINIADRFLSQHTNLFSFPVCKSKKDENVYEIDIAEGKELEGQDEVKKAKKPKGGKRLNGAVVKTFGSTKIMFNGIVDKNKKGQIKTKTRVYNIDGEWGGKTQKDEYVDKIRKVVDAMSPEEKAKVKAALKKCFSSSRADPKKKRKV

SEQ ID NO: 58 - protein, 970 aa, synthetic construct
MGPKKKRKVMDYKDHDGDYKDHDIDYKDDDDKMTKELSGVRVIELKTDLRKDQFWDRYERCFKTYHALYNEVPCWGLDWVEQKTQNQTSRELGCERVDLTAQRKALYERTDRTISYEQFSNCLKALWLGLLNCQQGNHMYTKLFEGAIQTDQMTAEDWAVLTEYVADPKSHNSQFLFRVSNTLKHIGFFSRPPFTATLFAPERKAITKDVMSDLKGWIEMKRMTEESYAAEEVQIQQMKAEVPVRIRQSLLRFFDTCIGLNLIGHFDERVHHYLRDCIIPALQQRTIPTEHFYLKSNRKDVGQKHIDFSLDIKFYELLAEMPELWNTLETSEDDLIPKPLILKHLHLLEAIMSHRAHRKTAAYAFVGEADYHRFYYLLGGNYTKHLISATGSELPDRVIWDNDKDVLMRNGRKVERLYVKVGDRKENFNFEVYTIAMNTKGLRGHRSTLKPTSYLQDLQIWSNPEGESTYLNFVRKGTERSAICKEPVLVYRNGAFFLRLSMSVEGMRASEEHIALQYYLSAAATGSDLSKDTEKTVERFNLIQGKTYKVMSVDLGIRSPFAWAVTESTITGVANPSQILNSGEMEIADDPDYTELFYAYKNLGHLIGQVKSSSKGKGLKADSHLVDMIHTVQRFFADYKVAGQRRSQIFEQFSKDPDPLYQMDQMMKRYENNLESVKKDFSFLINILFKYVTLQFGALRNRRRSYLSQNQMADQKFDQDFKWLNILEQRKRVTRSLSYLGTDNSRIPICLEQQKLDYNGCKDNFLKQLASKIVRIAHQNDCCLIVLEDLEGYGKTLNQRDENFLTAFWSPKRVKDAIINAAQWYGIGVVTVSEAQTSQVHHESGRIGYRKGRDLFFLTPDGQIESVPSDINAAKNIGHRFFSRHTDLHQVYLKGSDEGAKRMKGCLLYQFGSLEAARTHLTGTGPTWYLDGVEWIDKTERNLRRDLLKQRVEIEKMPFSRADPKKKRKV

SEQ ID NO: 59 - protein, 943 aa, synthetic construct; identical to SEQ ID NO: 56

SEQ ID NO: 60 - protein, 978 aa, synthetic construct; identical to SEQ ID NO: 55

SEQ ID NO: 61 - protein, 939 aa, synthetic construct
MGPKKKRKVMDYKDHDGDYKDHDIDYKDDDDKMKKPKQNIEETDLKITTPKTATIKATNLDDKMRLFTFFNGFTTVCSKVKDDIYNFGQNEDTLPVYTDYIKASQRARMCATTLATKSECDFAKKYGEHFPLPHYNQEGMNYTTHQHTYSVNSAVHTQLDSLNECDKLTNGEYVKLKKTVDELEEKLTEEHGKEPLDFLVKFVDEQILLGWRFDGKFRLFFEVAMLPELKNGNIIYKKAYKTSGGKGRRYSFYNPSVADNISKNPTVWNLLSDVKAVDYISLSNSLLRKKPHAQYTNTTLNRAQVRPTFGNNGVPFSISVSDDDYVYIRFRLPKKDGEEKGQEISVKCSYKTSYKGKRSKTLRKSCYLGNLKIEENGKGKYICKYNINGRETTTAELNECFLRVRINNNRWFNKYLNGTLTKEDGVLKSEYFDFYFDLCLNVHQKSIHGLTNSEIFGGKGKSIRSYYSTSYPEVKNLDGQKNIKTDFGCYVDKPHNIMGIDLGQRNPFAWAVLDQNGNVKDVGHLDGAENDTYKDYLTFSNRCKDVKNLILQSRDYLYGDDEAIDETLFDSVVQFVNSNITLNKYKSYLDEKKSLINKESLEKNRLYELKKKDHGWFVRDCLWFLTKEYHRINSERKTHSDWRYTLYWVDAIHRFIDVNKSFNSLGSYYDKKQSKSINGIQKDFCRSYWNQIDNLNEDTLKKFVFELLPVIKKNNVCLIAIEELKSMLGDDDKRAEDNRLYNLWPVGQLKTFLEGKLLPYNVAVMEVSEQNTSQIVNGQWSYREGDDLYYVKNNDNNTMCKTHADENAAINIALRAYSHHTNLYSIYMINPIDDYYVPSCIWNNKDEGSKRIRGFLTKTYGTSDVVFIKKNEKLVKSDVSIKDVKRIVKNIGNEKNKKSEIWYRMNDIEWIDEGSRDIIINTIKSKVRSRADPKKKRKV

SEQ ID NO: 62 - protein, 930 aa, synthetic construct
MGPKKKRKVMDYKDHDGDYKDHDIDYKDDDDKMTDKSISFKQFSQILNVLYKCIVISGKGRGLTSIILGQPQCKDSLTSADWGNLETLSAKDELTPAEVKDITKDLMYRASNTLVSIGFRNRSPFKLTLTSGERYAVVENVHRSLKSWVEVDKITRENYLNEEIALSDAFNNIDETLLPTLKEFFDACMNENIIHHFDARVYAYTRDCVIPALVAGLEIKDHFYIDGRDKAKRDYSLQGYAELLKGFPKLWQGVDPEILAKLYILEAQMDHKKHRPCAAYAFIGEDSYSRVQYLLGNNYTSFSPYALGVDLDDVTCGDDAEADTQFPKNKVIQFSQGKKVTKLSLTVSRGKEDTNKYSFDVFLADKYSNGSYKPSPYFSDLSVWVSEIGMLMEFTRKGERVQAIVKEPSLIYRKGAFYVRLNMGVIQDTSPEINDLYWYLSSGAPMSMTDRSKASETPKNTERLESIKGKSYRFLGIDLGLRSPFAWAVGEASISGVINKPTIIATGDYTTARDTRYDTLFFALKNAGKVIGVTKSLANGKDASFNGLMGTITAAREYLAHYSGVATHKVAAIQAFCQDDNPLETLKGLLKSYNNDLVTLKKDPRFIGGILLRYARLLKGELVTSRKMHLREHSVESKFGQEYMWLNILEREKRVCRSLSYLGLGNDRDSVIMGNLTTPYNHCKENLLKQLAARIVSLAVENKCHVIVMESLGGSNKSMNTRGQNFLEAFWSPQKIKDTIINAAAWHGIMVAEVSESQTSQVCFETGTFGHRDRASLYFLDKNGDLQETHADMNAAKNLVERFTTRHTNLRQVNMDSLPKEGPDKTPKKSPSKKKMEKAKMDNPEDQSKRLKGFLTVKFGNVKAAQEYFASRKPEQSYSGKKDEAIYWYLDGDEWITKKEKESRVSVIEGLVGLKEVAVSRADPKKKRKV

SEQ ID NO: 63 - protein, 864 aa, synthetic construct
MGPKKKRKVMDYKDHDGDYKDHDIDYKDDDDKMAFQSKRRIVGNLVKEQCLKAVDGKVILTDQEKRELIKRYELHLEPYKWLLRLFLSGYEGRDDGFYEELGNTNLDKEKFFEVTAGLRDALLRQSGSSRALKSSMLGKCPPSAAVGKAAKHIQALRDAGILPFKTGLTSGEDYNVLQQAVQQLRSWVACDHRTREAYAEQQEKTSQAEEAAKKAVNEVKPEDAKSLERHERALTKLRKQERRLERMRSHAQFSLDEMDCTGYSLCMGANYLKDYCLEKEGRGLRLTLKNSTMAGSYYVSVGDGQHAGMKNPGTPAGGSPEKGRRRNILFDFAVEKCGDNYLFRYDENGKRPRAGVVKEPRFCWRRKGNSVELYLAMPINIENSMRNIFVGKQKSGKHSAFTRQWPKEVEGLDELRDAVVLGVDIGINRAAFCAALKTSRFENGLPADVQVMDTTCDALTEKGQEYRQLRKDATCLAWLIRTTRRFKADPGNKHNQIKEKDVERFDSADGAYRRYMDAIAEMPSDPLQVWEAARITGYGEWAKEIFARFNHYKHEHACCTVSLSLSDRLVWCRLIDRILSLKKCLHFGGYESKHRKGFCKSLYRLRHNARNDVRKKLARFVVDAAVDAGASVIAMEKLPSSGGKQSRDDNRIWDLMAPNTLATTVCLMAKVEGIGFVQVDPEFTSQWVFEQRVIGDREGRIVSCLDAEGVRRDYDADENAAKNIAWLALTREAEPFCMAFEKRNGVVEPKGFRFDIPEEPTREQDESNQDFKKRLEERDKLIERLQAKSDRMRAIVRRLFGDRRPWDAFADRIPEGKSKRLFRHRDGLVLNKPFKGLCGSENSEQKASARNSRSRADPKKKRKV

SEQ ID NO: 64 - protein, 997 aa, synthetic construct
MGPKKKRKVMDYKDHDGDYKDHDIDYKDDDDKMDTDTELSDEVELSDEVELSDEVELSDEVELTVKKVKTTTVKVDNNFKKELFELFNHFTSVASGIKDRLYDLQFDENTASIFKGYIKEAKRGHGAATTVFTKLNPKKIYSGKKSFPRDYRDRGIFPFYNKESGKYDLSTCGYHYSANAEIHTQLNSHDECNKQCEKEYAALEKERNKYKHEFTRQFKAENVEKFSNFVEKLTLMGWRYDATFRNFFELHMHPKLKTSETTYRATYKLPSGKSKRYSFSRDDIADEIAKNPEFWPMLESSNAVSWINSNNLLSRKKEKANYSSTSLIKSQIRLYLGDNGVPFTAREHDGRIYFSFRLPSINGEKGRNVEIPCSYKKVFNGKARKSCYLGGLTIENTGGSKHIFKYSVNNKKPQVAELNECFLRLVVRNHGYFNKMVNGKLTDKDGKLHADYFDFCIDLPLNVKEDPIHDLTYQEINGVKANPEKNIEKKVGLLGFYQSAYPEIKNLGSQIETGKNLTCPITKTHNIMGIDLGQRNPFAYCIKDNNGKFIAKDHMDGSKNETYKKYINFGKESTSVSHLIKETRSYLHGDPEAISKELYNEVSGLCNSPLSYEEYLKYLDSKKFLINKEDLNKNAMHLLRQKDHNWIGRDWLWYISKQYKKHNENRMQDADWRQTLYWIDSLYRYIDVMKSFHNFGSFYDKNLKKKVNGTAVGFCKTIYDQINNNNKDMFKKFTNELIPIIRKHKVSVVALEKMESMLGDKSRNTFENRNHNLWPVGQLKTFIENKLDGFNVIVVEVDERNTSQMCDGNWSYREADDLYYVKDGELREVHADENAANNIVDRCISRHTNIFSLYMTNPMDDYYVPACIWDRSENGKRGRGFLTKMYKNSDVVFTKKDDKLVKSKMSVKELKKLVDKTKEKRGQYWYLFEGKSWINAADRDTIISNAKKLFRERDGGEQSTDTRSQNVTVSVLDVCETVEKKKLVLVSRADPKKKRKV

SEQ ID NO: 65 - protein, 1044 aa, synthetic construct
MGPKKKRKVMDYKDHDGDYKDHDIDYKDDDDKMSTEVDVKTINLKIAKKGGVYPILEQSIKENCKSNDLLEFFMVLNRLQTYYIESNEEILVDFPKKYDELFDIVKNNDSSVTREYFDSLCDKYITEVCANGFVNNVYIAHNKNQELNWAETSNDRKIKSNKTFMFGKIKGLIRDKFGREELSDKDATKQLCEDIFNLFILNNANIELDEKYNIIKDELIQIWNERNKEFIHIKDITLLFRQWGILPTYDNITHNCELKAIIAEPVRRFKSWLECNSEANKNYDTEREKCTKYMDVMDSDLTVEFSKMVTELGNPFGANDKNIYKYFNQKFLLFFKQVVQPKFVNGEPLDESNGSYSGEIKINSAGKVENYSIAVSVIDTIKKYPTIWSDRSWGESVISTVAKIDPQYGIDDITDDMQVSPFYLFYGYFTAYNYIQQHKRNAKYTPISKDSLPSLYLGNNYIPFKIDCENVDDDRFYITIKNMNNLKLNVLYRKPKLKFAKTKEKTKRNKCYFDNLKITNTNNNFKFEYNINGDPNRSVVAYLKEPVIRYNNRKDYFYLSATISKDVETDSELTSACWSKISNDTARRVNAEQYFNDNGVNIVGIDLGMNPIIAYSVLHYKNNEFIDLNITGKIADKDKHPNLNYKRMYEKRSEIKKLKTLIKMIPDYVNSDSNIFEGDNNVFKQLDKKSKGRFRSSEYMGYYDKLNVDGKFISELEIVKKVVNTKHYKNDTEKNNDIMRVYKGNKKNIIKKEIDTHRHQIHSIKDMNRRSDESNLCYVYDMVSYIDDFKKLVTSYNKIGEDYNNPIKPLSDPMLFSKSKLYEYRQNIRDNFLKDICYQMVKIAKQYNAVLVHEHFEQRKGGIDRVNNILMALFTPNDIIKKLKCVAKREGVLVFNTNKNHTSQYVYNKNTVGYRDSNNKHNLYYIEDETTRKLGVVDSDINASKNIAARPFNKPLYAIKVKNYDDGLFLSDYNNKYVLYKKDGDKYVAIGDTYRIDKKKIKQGSVTLYLHNGYYVDGEYKNNYIENIKKLVLSRADPKKKRKV

SEQ ID NO: 66 - protein, 864 aa, synthetic construct
MGPKKKRKVMDYKDHDGDYKDHDIDYKDDDDKMAFQSKRRIVGNFVKEQCLKAVDGKVILTDQEKRELIKRYELHLEPHKWLLRLFLSGYEGRDDGFYEELGNTNLDKEKFFEVTAGLRDALLRQSGSSRALKSSMLGKCPPSAAVGKAAKHIQTLRDAGILPFKTGLTSGEDYNVLQQAVQQLRSWVACDHRTREAYAEQQEKTSQAEEAAKKAANEVKPEDAKSLERHERVLTKLRKQERRLERMKSHAQFSLDEMDCTGYSLCMGANYLKDYCLEKEGRGLRLTLKNSTMAGSYYVSVGDGQHAGMKNPGTPAGGSPEKGRRRNILFDFTVEKCGDNYLFRYDENGKRPRAGVVKEPRFCWRRKGNSVELYLAMPINIENSMRNIFVGKQKSGKHSAFTRQWPKEVEGLDELRDAVVLGVDIGINRAAFCAALKTSRFENGLPADVQVMDTTCDALTEKGQEYRQLRKDATCLAWLIRTTRRFKADPGNKHNQIKEKDVERFDSADGAYRRYMDAIAEMPSDPLQVWEAARITGYGEWAKEIFARFNHYKHEHACCAVSLSLSDRLVWCRLIDRILSLKKCLHFGGYESKHRKGFCKSLYRLRHNARNDVRKKLARFIVDAAVDAGASVIAMEKLPSSGGKQSKDDNRIWDLMAPNTLATTVCLMAKVEGIGFVQVDPEFTSQWVFEQRVIGDREGRIVSCLDAEGVRRDYDADENAAKNIAWLALTREAEPFCMAFEKRNGVVEPKGLRFDIPEEPTREQDESDQDFKKRLEERDKLIERLQAKADRMQAIVQRLFGDRRPWDAFADRIPEGKSKRLFRHRDGLVLNKPFKGLCGSENSGQKASARNSRSRADPKKKRKV

SEQ ID NO: 67 - DNA, 2805 bp, synthetic construct
  source 1..2805: mol_type = other DNA
atgggacccaagaagaagcgtaaggtcatggactataaagatcacgacggcgattataaagaccacgacattgattacaaggacgatgatgacaagatgagcaactacaaaaacattaagttcaagttggttccgttcagtcaaaaggatcttataaacatgcagctaaacgtgaatctccaccagcagtgttatagagagttcgtggagcagttctgcgtcctctgtaatatcccctttcctgggcttagtaaagatcaaattgagcagaagcggaaacaattaaatctgtctgaagacgacgagaaggacatcaactacatcaaggaccttgtaaaaaataagaataacatcggcaattcaatctatgcttttttcactggtacaaagaaggaaatgccaagcagaaagactgatttaacacctctttaccgcctccttaaggctaacatactgccctttagcctcctcaaagggcgagagaactataagaaaagcatattccaaactgttattaaccagacactggaaaagtttaagtcatatttcaagtgcaatgaatcagttgaaaacaacttcaaactgtctctgaacaaggactcaaatgaggagcaagtcctgaatgaaagcgaaatgaaagacctccaaaacctattcgagaatttgtctaaaaatcagtctttttccttcttcaacttcaataagaactggttctccaaggacaagatcaagacgaaactcctcaataacgagaccaacaaaattaagtcgttgtcatctgaagagatcgacctgatccttagttataaggataagttgtactccaacgaatttgatctgatttccatgttcgtggagttcaacttacagaaacagaaggcggagtccttgaaatcacaggcggacttgaacctcttcaagaacaacaactattcttttcggattggaagcaactatgaaaactttaatctaactcaaaataacaaggacatcctgctggaaatcaattcttcaatgggtgagaagattacctttaagatcattccgcataagaaaacccagatctggaatttagagaagaataatgttaagataacttcgggcgagaacctggggaattacaaatcggtggacgtcatcaagatgaagcggccagcagacattaaggcaaagctgctgaagacgtcagagctgaatatcgagatcaagaacaaccaaatctattgcaacttcatttatgagtacaagtgctccgatcatggcgtgtacttctttcactgcagtggcaacaagaagccagatgagaagaatgagaatattctaaaggagagggagaggacctttagtttcattgatctcggtctttttccgatgtattccatctccacatttaagtacaataataagagcaatgatggtgagatcctagtcaagtcgggatctgggaacgagaaactcgacttcggctctgccttcaaaattcattcaatccagattggaaagaacagcacaaatctcaacaaaattaagcaacttcttgagaagctgaaagacctgaagacctacctcaaattctctaagagcataagcagcttcgacgagaacagctaccagcgccagcttaaaacgggagtggagatcagcgagctgaacagcctgtcgttccaaaaaatatcagaaattaagtccattaatctcggcttcaatgaatccttcaataaagagtattttctaaagctgatcgaaaaccaaacattcacgcagaaggagttactactgttaaactgcaagatcaaagacctcttcaaaattctctacaaagaatattctaacatcaaaaacagtcgcatatttaaattcaataaagaagatgatctcatctgtgacgggtactactggctgcaggtcattgatgaaataatcaatattaaaaagtcgcttacttacttcaacagcaagccgtcggagaaggggaacaaaagtaagtttattttcttgaaggattttaactacaaaaataattttgcaaacaactacgcgaaaatcgctgcgtcacgtctcaaaaaatattgtttggagcacaaggttgacgtgtgtgtttttgagaagaacctcaacaactttctgcaaagcaaggacaacgataaaaagacaaataagaccttgattaattgggcgaaccgcaatctttttgagaaaattaaattggcgctggaagagcatgacatctgcgtgagtgaggttgatggtaagcattcgtcccagctggacccgcaaaccatgaactggggcgctagagataatcttaatggaaatggtaacaaagaaaagatcttttttgaaaggaacgggcagataatacaacagaacgccgacctcagtgcttctgaagtcctcgcaaaacgattcttcaccaggtacgaggacatcgtgcacatctacattgaccagaaaataaaggatgacaaaacgatccttaagttggtgaagggtaaggtgcgcgtagaatcttatctgaagaagactataaattcctgctacgccatagtagatgaaaatggcttccttaaacctatatctaagaaagactacaacaagttccaggagctgccgtccaagcctcgcacagatattaagtcgaatgagatgtacagacatggcagcaagtggtatcacttccagcaacatagggagtttcagcaggacctgttggcacggggcagagagctgaagaagatagccggcagcggcagtaaaaggccagccgccaccaagaaagccggccaggctaaaaagaagaagtga

SEQ ID NO: 68 - DNA, 2964 bp, synthetic construct
  source 1..2964: mol_type = other DNA
atgggcccaaagaagaagaggaaggtgatggactacaaggaccacgacggcgactacaaggatcacgacatcgactacaaggacgacgacgacaagatgaacaagacggacacccagaacaacgagcagatcaacaagccgacgcagctgctcaacaacaaggacattgagctgacggtgaagaccgtgaagtccgcgaccgtgaaggtggacaacaacagcaagaaggagctgttcggcctgttcaactacttcaccagcgtcgcctccggcatcaaggacaaggtgtacaacctgcagtccgatgagaagaccgccccgatcttcaacgactacgtgaagcagccgcagcgcggcaggtctgctgctactactctgttcaccaagctggacgcggagaagacctacacctctcagcactccttccccggcaagtggagggattccggcatcttcccgctgtacaacaaggagtccgagaagtacgacctgtccacccacggctaccactactccgctaacgccgagatccacacccagctggacagccatgacgagtgcaacaaggagtgcgagaaggagtacgccgcccttagggacgaggtgaacaactacaagtacgagttcacgcttcagttcaaggccgagaacgccgagaagttctacaacttcgtggagaagctgacgctgatgggctggaggtacgacgctacgttcaggtctttcttcgagctgcacatgcacccaaagctcaagaccggcgagacaacgtacagggccacctacaagctgccgtccggcaagtctaagaggtacagcttcttcagggacgacatcgccgacgagattgccaagaacccagagttctggccaatgctggagtcctccaacgccatctcctggatcaactccaacaacctgctcagcaggaagaaggacaaggccaactactcctcaacctccctcatcaagtcccagattcgcctgtacctgggcaacaacggcgtgccattcaccgctagggagcacgatggcaggatttacttcagcttcaggctcccggccatcaacggcgagaagggcaggatggtcgagatcccatgcagctacaagaaggtgttcaacggcaaggccaggaagagctgctaccttggcggccttaccatcgagaagaccgacgctggcaagcatatcttcaagtactccgtgaacaacaagaagccgcaggtggccgagctgaacgagtgcttcctgaggctggttgtgaggaatagggagtacttcaacaacgtggtggccggcaagatcaccgacatcaacaccgatcacttcgacttctacgtcgatctgccgctgaacgtgaaggaggacccgatccatgatctgagcagcacggaggtgttcggcaagaatggcctgaggtcctactactcctccgcctacccagagattaagaacctgggctcccagatcgagacgggcaagaacctgacctgcccgatcaccaagacacacaacatcatgggcatcgaccttggccagcgcaacccattcgcctactgcattaaggacaacaccggcaagctcatcgcccagggccatatggacggctctaagaacgagacgtacaagaagtacatcaatttcggcaaggagtccacctccgtctcccaccttattaaggagacgaggtcctacctgcacggcgatccagaggctatctccaaggagctgtacaatgaggtcgccggcttctgcaacaacccggtttcctacgaggagtaccttaagtacctggactccaagaagttcctgatcaacaaggaggacctgtccaagaatgccatgcacctgctgaggcagaaggaccacaactggatcggcagggactggctgtggtacatcagcaagcagtacaagaagcacaacgagaacaggatgcaggacgccgactggaggcagactctgtactggatcgacagcctgtacaggtacatcgatgtgatgaagtccttccacaacttcggcagcttctacgacaagaacctgaagaagaaggtgaacggcaccgtggtgggcttctgcaagacggttcacgaccagatcaacaacaacaacgatgacatgttcaagaagttcaccaacgagctgatgagcgtgatcagggagcacaaggtgagcgtggtggcgcttgagaagatggacagcatgctgggcgacaagtcaaggcacacgttcgagaacaggaactacaacctgtggccggtgggccagctgaagacattcatggagggcaagctggagtccttcaacgtggccctgatcgagatcgatgagaggaacaccagccaggtgtgcaaggagaactggtcctacagggaggcggatgacctgtactacgtgacggacggcgagtcccacaaggtgcatgctgacgagaacgcggccaacaacatcgtggacaggtgcatttccaggcacaccaacatgttcagcctgcacatggtgaacccaaaggacgactactacgtgccgacctgcatttgggacaccacggaggagtccggcaagagggttaggggcttcctgaccaagctctacaagaactccgacgtggtcttcaccaagaagggcgacaagctggtgaagagcaagacctccgtgaaggagctgaagaagctggtgggcaagaccaaggagaagaggggccagtactggtacaggttcgagggcaagagctggatcaacgaggccgacagggacaccatcatcctgaacgccaagaagatctccagggaaagggacaacggcgagcagtccacggataccaggagccagaacgtgaccgtgtccgtgctggacgtgtgcgagacagctgagaagaagaagctggtccttgtgggcagcggcagcaagaggccagctgctactaagaaggccggccaggctaagaagaagaagtga

SEQ ID NO: 69 - DNA, 2859 bp, synthetic construct
  source 1..2859: mol_type = other DNA
atgggcccaaagaagaagaggaaggtgatggactacaaggaccacgacggggactacaaggatcacgacatcgactacaaggacgacgacgacaagatgaagagcataaagagcataaaaagcatcaagacgaaggtggtgaagaacaacgagctgaagctgatagagctgagtacgtggtgcagcagcatatgcgagcagctggagaggtacatattcatcctgggggggaaacaaatacacgacagggacggcgtggtggtgctggacggcgcagtggagaggaagatctactgtaagaaagacaagagcttgatcgcggcctgcgaggtggtgtacaaacacttcacggacaagagttccaagtccaggacgtttgggtcctggttcctgggtgggaagtccgagggcgacaacaccaataagggaaggaagagtaccaaggagaagaccgagaaacaaatcgcaaagcagatcgccgacaagaaggagctgacggactccctgcaactgctgtgggacaagaagctgctgccattcccgatagacaacaagggctacgacttcataaataccccaagggccaaatcctacaagtgggcgatcacgaaaaccatccacgctaaaatcaaatcctacaacgagcaatgcgtggagaccaaaaaagagtacgacgccctgaacgccgagatcaacacctacaagaccatcctgttctccggctactccgaaaaggacatcgacgacctgcagaagttcgtggacatctgcgaggcaaacaaccacaggataaactacaaattcatatcctttctcaagaggaaagacctcaatttcgacgaacaaacagggaaatacaggaaggaaggcaagtggattcaacacaagaacggaaaggaagtcaagagcaagtacagcatgaaggacgagatagtggaggccctgtacaagtacaagtccctgacaaagaacgacgtgagcgtgctgtgcaacgagcaccaaaaagaggacgaaatgggcaaggtggtgcattacaacatgaagaggtactctgatctgctgttcagaaagaagaacaaaaaggaaatcccgagttacacgaaaatcagcctggccaccagcaagattgagttggggttgaacaatgtgaagtacaacgtggagcaggtggaggacaaactgatatggaccatatgcgaccagaccggcaaggacatccagttcgtgaccgtgtacaccaggaagaaggaggataacaggaccaatggcaagaaaggggcggggttctacaagggcaaacaccaccagctggaggacctgaaaatagtgccggtgggcgacatagggacctacgacatcagcttcaaggtgaacgggaagaggccgttcacagggaccctgaaggaaccgaacatcatatgcaggggcgggaaggtgttcgtccagatgccgatcaacatcaacatcgacaaaaccctgaacgacgcgaggaagaaggtgctgtacgcataccgggagacgtactccggctccgtgaacggcaagaagcagaagatgataaagatcgaaaactccaaaatcgccgagtccctgaaatccctggggcgggacgcgatagtcctgggcgtggatctggggctgagggggctggctacagcggtggtgagccacaacgggaaaaacgagacagtgaagagcagccaatacattaagggcgacattgtggagtgggagaagtacagggtgtttaacgacaacatcagggaggtgaagaagtacatattcctgaccaagaagtcctataccgccacgacggaggaatacaccgagttttacaaggagtgctcgaagccggagcaggactatctggactccctcaagacctataaagacaagaacgtgaaactcaacgagctgaaatacacgaagaacgcgtggtccgtgagcaagatgttcgaagacgtctccaaaatgttcgaaaccctcaagcaggacaggctgaagtactacgacatcttcaacatgccatactgggccgcctccctgaagaactacatgagcctgatgaagtcctacaactacgtcggcgtggacataaaggtgtccaaagaatacatgagcaagtaccagtccctgtacaacaacatcaaggaagattacgccaaaaaaatcggctcctacatcgtgcagctcgccgtggccaagaattgcgacatcattgtcctggaggagctgaaatccaacctcggctccgtggacaggaagagcaagagagacaacgagatgtccctgatgtggaactgcggccgcatcaagacccacgtcgagaacatggcaaaggactatgggatgttcattgacgaagtcccggagtatggcacgtcccaggtgtatcacaagaccggcaactacggctacagggatgaagacaacagggagatattttggtacgaggacaacaaggacgtggcctacatacacgccgacgagaacgcggcaatcaacatagccaaaagattcctgtcccaacataccgacaactccagcttcagcgttatcctgaagggcgacgcctactacctgaacatcgcctccaactccaaacgcatgagggccgccgcactgaaaaccttcggcgacctcaacaaaccgttcaaaatcaacgccaacgacaaaaacggaaacctgtacaagaagaccaggatcttcaagtccgactccagatggataggcgtcaacgacaaagacctctacatagaacacatcaaatccctccgcaacctccgcgtgcgccagggttccggttccaagcgcccagccgccaccaagaaggccggccaagccaagaagaaaaaatga

SEQ ID NO: 70 - DNA, 2040 bp, synthetic construct
  source 1..2040: mol_type = other DNA
atgggcccaaagaagaagaggaaggtgatggactacaaggaccacgacggggactacaaggatcacgacatcgactacaaggacgacgacgacaagatgccgagcttcacgaaggtggacgaggacaaaatagtgctgaagctggggaacaactacatcccgtatgggctgagcaggatttccgaggacaagatgctgtggagcttttcctccccgcaaaaaaagaagctgtctataataacgaaccacaggcgcgtcggcaagggcaaacacttttacctggaaggcttggagatcgccgacattaccaagggcgacggcgacaagacgtccccaagcggcaaatataccatctccttcagcatcaacggcaagcaggacgtgaagggcgagctgaaggagccgagcttcggcctgaggaacggcaacgtgtacatgtttctgccaatctccataaagcagaccgacgtgttcgagtccagggtggagatgaggaggttgctgtctatggcctaccagccaaccaccgtggaggatctgatcctggatgacgtggagaccaagcagaagaccgtgaagcaggggaagaaggaggtgaacaccacgaacatagcgattcaagaggcgatcaagaagcacggccgcctgctgaaggtgatgggcgtggacctggggctgaggaacttcgcgtttgccatcaagaactacgacggccaccacgacaccctgttgcggcagttgtactccgagtccgacctgaacgagaaacagaggtacactaccctggccaatgacttgtccaaggtgggcaaccacatcaagttcgccgcggtcttctacggcgccaacgacaccgaggagaacaccaagatgttcgacgccgagtgcacggacgccgagtccaggacccacctggagtggctgaggaaagccaagaagtccggtgtgctgctcaaggacctgaggaaggacaagacgtggatcgtgtcgatcaagtataccgagttgaggaataggctgcacgcactgaaattcggcaggatgaagagctacgactacaggaataacctctactgggccgcgaccattaagaagttcatctcgctctccgccagcttctacggcgtggggaggcctagccgcggcaagaaggacgtgagggagttgaagaaaaagcacaccttcttctccacgtatcaggacctgtacaacaacgtgaaggaagattacgcgaagaaggtggcgaatctggtggtgatgacggccaaagagaataacgtggacatcatcgtggtggagaacctgaccgggcactgcgggtccaaggactacaagaccagggccgagaacgagatgagtataatgtggaatcatggcaggatcaagacgttcatcgattgcatcgccaatgccaacggcatgttgttggccgaggtgtccgagttcgagacgtcccaggtgtaccacgagacgaggaactacgggtacagggacaagaagatgaaagagatcctgtggtacatggactccgaggggaacgtgcagtatgcccacgccgaggtgaacgccgccatcaatatcgccgacaggttcctgtcccagcacaccaacctgttctccttcccagtgtgcaagtccaagaaagacgagaatgtgtacgagatcgacatcgccgaggggaaagaacttgagggccaggatgaagtgaagaaggccaagaaaccgaaaggcgggaagaggctgaacggggcggtggtgaagacgtttgggagtaccaagatcatgttcaacgggatagtggacaaaaacaagaaggggcagataaagacgaagacgagggtgtacaacatagacggggagtggggggggaagacccagaaagacgagtacgtggacaaaatcaggaaggtggtggacgcgatgagcccggaggagaaagcgaaggtgaaggcggcgctgaagaagtgcttcagcagcggcagcgggagcaagaggccagccgcaacgaagaaggcggggcaggcgaagaagaagaagtga

SEQ ID NO: 71 - DNA, 2940 bp, synthetic construct
  source 1..2940: mol_type = other DNA
atgggcccaaagaagaagaggaaggtgatggactacaaggaccacgacggggactacaaggatcacgacatcgactacaaggacgacgacgacaagatgacgaaggagctgagcggggtgagggtgatagagctgaagaccgacctgaggaaggaccagttctgggacaggtacgagaggtgcttcaaaacgtaccacgccctgtacaacgaggtgccatgctggggcctggactgggtggagcagaaaacacaaaaccaaacctccagggaactcggctgcgagagagtggatctgaccgcccaacgcaaggcactgtatgagaggacggaccgcaccatctcttacgagcagtttagcaactgcctcaaagccctctggctggggctgctgaactgtcagcaggggaaccacatgtacaccaaactgtttgaaggcgcgatacaaaccgaccagatgaccgcggaggactgggccgtgctgaccgaatacgtcgcggacccgaagagccacaactcccagttcctgttcagggtgtccaacaccctgaagcacatcggcttcttctccaggccgccatttaccgccaccctgtttgccccagagaggaaggctattaccaaggacgtcatgtccgacctgaaaggatggattgagatgaagaggatgaccgaggagtcttacgccgcggaggaggtgcaaattcaacaaatgaaggccgaggtgccggtgcgcatcaggcagagcctgctgaggtttttcgacacctgcataggcctgaacctcatcggacacttcgacgaaagggtgcaccactacctgagggactgcataataccggcgctgcagcaaaggacgataccgaccgaacacttctacctgaaatccaaccgcaaagacgtgggccagaaacacatagacttcagcctcgacatcaaattctacgagctgctggctgaaatgccagagctgtggaacaccctggagacctccgaggacgacctcatccccaaaccgctgatcctcaaacacctgcacctgctggaagccatcatgtcccacagggcccacaggaagaccgccgcctacgccttcgtgggcgaagccgactaccacaggttctactacctgctcggcggcaactacacaaaacacctcatcagcgccaccggctccgaactgccggacagggtgatctgggacaacgacaaggacgttctgatgaggaacggcaggaaggtggagaggctgtacgtgaaagtgggcgacaggaaagagaacttcaacttcgaggtgtacacgatagcgatgaacacgaagggcctgagggggcacaggagcacgctgaagccgacgagttacttgcaagacctgcagatttggagcaacccggagggcgagagcacctatctgaacttcgtgaggaagggcacagagaggagcgcgatttgcaaagagccagtgctggtgtacaggaacggcgccttttttcttaggctgagcatgagcgtggaagggatgcgggcctccgaggagcatatcgcgctgcagtactacctttctgccgcggccacgggctctgacttgtctaaggacacggagaagaccgtggagaggttcaacttgatccaggggaagacatacaaggtgatgtccgtggatctcggcatccgctcccccttcgcctgggctgtgaccgagtcgaccatcacgggcgtggccaacccgagccagatcctgaacagcggcgagatggaaatcgcggacgacccggactataccgagctgttctacgcttacaaaaacctggggcacctgatcggccaggtcaagagcagcagcaaggggaaaggcctcaaagcggacagccacctggtggatatgattcatacggtgcaaaggttcttcgccgactacaaagtggccgggcagaggaggagtcaaatattcgagcagttcagcaaggacccggacccgttgtaccagatggaccagatgatgaagaggtacgagaacaacctggagagtgtgaagaaggattttagtttcctgataaacatcctgttcaagtacgtgaccctgcagttcggagccctgaggaaccggagaaggagctacctgtcacaaaaccagatggccgaccagaagttcgaccaagacttcaagtggctgaacatcctcgagcagaggaagcgcgtgaccaggagcctgagctacctgggcacagacaacagcaggattcctatctgcctggaacagcagaagctggactacaacggctgcaaggacaacttcctgaagcagctggcctccaagatcgtgaggatcgcccaccaaaacgactgctgcctgattgtgctggaggaccttgaggggtacgggaaaacgctcaaccagagggacgagaacttcctcacggccttctggtctccgaagagggtgaaggatgccatcatcaacgccgcccaatggtacggcattggggtggtgacggtgagcgaggcccagacgtcccaggtgcaccacgagtccggcaggatcggctatagaaaggggagggacctgtttttcctgaccccagacggccagatcgagtccgtgccgagcgacattaacgccgccaagaacattggccataggttcttttccaggcacaccgacctgcaccaggtgtacctgaagggttccgacgagggcgccaagaggatgaaaggctgccttctgtatcagttcgggagtctggaggcggcccgcacgcaccttaccggaacaggaccgacctggtacttggacggcgtggagtggatagacaagacggagaggaacctgaggagggacctgctgaagcagagggtggaaatcgagaaaatgccattcggcagcgggagcaagaggccggccgctactaagaaggcggggcaggccaagaagaagaagtga

SEQ ID NO: 72 - DNA, 2859 bp, synthetic construct
  source 1..2859: mol_type = other DNA
atgggaccaaagaagaaacggaaggttatggattacaaagatcacgatggcgactataaagaccatgacatcgattacaaggacgacgatgacaagatgaagagcatcaagtcgatcaagagcattaagactaaagttgtcaagaacaacgagctgaagctcatcgagctgtctacctggtgtagctcgatctgcgagcagctcgagaggtacatcttcatactgggcggcaagcagattcacgatcgcgatggcgtcgttgttctcgatggcgccgttgagcggaagatctactgcaagaaagacaagagcctgatcgccgcctgcgaggttgtctataagcactttaccgacaaatcgtccaagtctcgcacctttggcagctggttcttgggcggcaagagcgagggcgataacacaaacaagggcagaaagtccaccaaagagaagactgagaagcagatcgctaagcagatcgccgacaagaaggagctgaccgattctctgcagctcttgtgggataagaaactgctgccatttccgattgataacaagggttacgacttcatcaacacaccacgcgccaagagctacaagtgggctatcaccaagaccattcacgcgaagatcaagagctacaacgagcagtgtgtcgagacgaagaaagagtacgacgcgctgaacgccgagattaatacatacaagactattctgttcagcggttactccgagaaagacattgacgacctccagaagttcgtcgatatatgtgaggccaacaaccacaggatcaactacaagtttatcagcttcttgaagcgcaaagatttgaatttcgacgagcagacaggcaagtaccgcaaggagggcaagtggattcagcacaagaacggcaaagaagttaagtccaagtacagcatgaaagatgagatcgtcgaggcgctgtacaagtacaagagcctgactaagaacgacgtgagcgtgctctgcaacgagcatcagaaggaggacgagatgggtaaggtggtccactacaacatgaagcgctattccgacctgctgttccgcaagaagaacaagaaggaaataccaagctacacaaagatctcacttgccacgtccaagatcgagctgggcctcaacaacgtcaagtacaacgttgagcaggttgaggacaagctcatctggacaatctgcgatcaaacaggcaaagacatccagttcgtgactgtctatacaagaaagaaagaagataacaggaccaatggcaagaagggagcgggcttctataagggcaagcatcaccagctcgaagacctgaagatcgtgcctgtgggagacattggcacttacgacatcagcttcaaggtcaacggcaagcgtccgtttactggcactctgaaagagccgaacatcatttgccgcggaggcaaagtgttcgtgcagatgccaattaatatcaatatcgataagactctcaacgacgctcggaagaaggttctgtacgcctacagggagacgtacagcggctccgtcaacggtaagaaacagaagatgatcaagatcgagaacagcaagatcgccgagtcactcaagtctttgggcagagacgccattgtgcttggcgtggatttgggcttgcgcggacttgctaccgccgttgtgagccacaacggaaagaacgagactgttaagagcagccagtacatcaagggcgatattgtggagtgggagaagtacagggtgttcaatgataatatcagggaggtcaagaagtacatcttcttgaccaagaaaagctacaccgccacaacggaagaatacacagaattttacaaggagtgcagcaagcctgagcaagactatcttgatagcctcaagacgtacaaggacaagaacgttaaactgaacgaactgaagtacaccaagaacgcctggagcgtctcgaagatgtttgaagacgtttccaagatgttcgagacactcaagcaagacaggctcaagtactacgacatcttcaatatgccgtattgggcggcctcactgaagaactatatgtcgttgatgaagtcgtacaattatgttggcgtggacatcaaggtcagcaaagagtacatgtccaagtaccaatccctgtataacaacatcaaggaggactacgccaagaagatcggcagctacattgtccagctggctgtggcaaagaactgcgacatcatcgtgcttgaagagctgaagtcgaacctgggcagcgttgatcgcaagtccaagcgcgataacgaaatgagcctcatgtggaactgcggcagaatcaagactcatgtcgagaacatggccaaagattacggcatgtttatcgatgaggtgcctgagtatggtacttcgcaggtgtaccataagaccggtaactacggctatagagatgaagacaacagggaaatcttctggtacgaggataacaaagacgtcgcctacatccatgcagacgagaatgctgccatcaacatcgcgaagcgctttctgtcacagcataccgacaacagctcattctccgtgattctcaagggcgacgcttactacctgaacatcgcttccaactccaagagaatgcgcgccgccgctctcaagacctttggagatctcaacaagcctttcaagattaatgccaacgataagaacggcaacctctacaagaagacaagaatcttcaagtcagactctcgctggatcggcgtgaacgacaaggacctctacatcgagcacatcaagagcctgagaaatctcagggtgaggcagggctcgggcagcaagaggccggctgccactaagaaggcaggtcaagcgaagaagaagaagtga

SEQ ID NO: 73 - DNA, 2964 bp, synthetic construct
  source 1..2964: mol_type = other DNA
atgggcccaaagaagaagaggaaggtgatggactacaaggaccacgacggcgactacaaggatcacgacatcgactacaaggacgacgacgacaagatgaacaagacggacacccagaacaacgagcagatcaacaagccgacgcagctgctcaacaacaaggacattgagctgacggtgaagaccgtgaagtccgcgaccgtgaaggtggacaacaacagcaagaaggagctgttcggcctgttcaactacttcaccagcgtcgcctccggcatcaaggacaaggtgtacaacctgcagtccgatgagaagaccgccccgatcttcaacgactacgtgaagcagccgcagcgcggcaggtctgctgctactactctgttcaccaagctggacgcggagaagacctacacctctcagcactccttccccggcaagtggagggattccggcatcttcccgctgtacaacaaggagtccgagaagtacgacctgtccacccacggctaccactactccgctaacgccgagatccacacccagctggacagccatgacgagtgcaacaaggagtgcgagaaggagtacgccgcccttagggacgaggtgaacaactacaagtacgagttcacgcttcagttcaaggccgagaacgccgagaagttctacaacttcgtggagaagctgacgctgatgggctggaggtacgacgctacgttcaggtctttcttcgagctgcacatgcacccaaagctcaagaccggcgagacaacgtacagggccacctacaagctgccgtccggcaagtctaagaggtacagcttcttcagggacgacatcgccgacgagattgccaagaacccagagttctggccaatgctggagtcctccaacgccatctcctggatcaactccaacaacctgctcagcaggaagaaggacaaggccaactactcctcaacctccctcatcaagtcccagattcgcctgtacctgggcaacaacggcgtgccattcaccgctagggagcacgatggcaggatttacttcagcttcaggctcccggccatcaacggcgagaagggcaggatggtcgagatcccatgcagctacaagaaggtgttcaacggcaaggccaggaagagctgctaccttggcggccttaccatcgagaagaccgacgctggcaagcatatcttcaagtactccgtgaacaacaagaagccgcaggtggccgagctgaacgagtgcttcctgaggctggttgtgaggaatagggagtacttcaacaacgtggtggccggcaagatcaccgacatcaacaccgatcacttcgacttctacgtcgatctgccgctgaacgtgaaggaggacccgatccatgatctgagcagcacggaggtgttcggcaagaatggcctgaggtcctactactcctccgcctacccagagattaagaacctgggctcccagatcgagaccggcaagaacctcacctgcccgatcaccaagacacacaacatcatgggcatcgaccttggccagcgcaacccattcgcctactgcattaaggacaacaccggcaagctcatcgcccagggccatatggacggctctaagaacgagacctacaagaagtacatcaatttcggcaaggagagcacctcagtctcccacctcatcaaggagaccaggagctacctgcacggcgatccagaggctatcagcaaggagctgtacaacgaggtggccggcttctgcaacaacccggtttcctacgaggagtacctcaagtacctggacagcaagaagttcctgatcaacaaggaggacctgtccaagaacgcgatgcatctcctgaggcagaaggatcacaactggatcggcagggactggctgtggtacatcagcaagcagtacaagaagcacaacgagaacaggatgcaggacgccgactggaggcagactctttactggatcgacagcctgtaccgctacatcgacgtgatgaagtccttccacaacttcggctccttctacgacaagaacctgaagaagaaggtgaacggcacggtggtgggcttctgcaagacggttcacgaccagatcaataacaacaacgacgacatgttcaagaagttcacgaatgagctgatgagcgtgatcagggagcacaaggtgagcgtggtcgcccttgagaagatggactccatgctcggcgacaagtccaggcacaccttcgagaacaggaactacaacctgtggccggttggccagctgaagacgttcatggagggcaagctggagtccttcaacgtggcgcttatcgagatcgacgagaggaacacctcccaggtttgcaaggagaactggagctacagggaggcggacgacctgtactacgtgacggacggcgagtcccacaaggtgcatgctgacgagaacgccgcgaacaacatcgtcgacaggtgcatcagcaggcacaccaacatgttcagcctgcacatggtgaacccgaaggacgactactacgtgccgacctgcatctgggacaccaccgaggagagcggcaagagggttaggggcttcctcacgaagctctacaagaactccgacgttgtcttcaccaagaagggcgacaagctggtgaagtccaagaccagcgtgaaggagctgaagaagctggttggcaagaccaaggagaagaggggccagtactggtacaggttcgagggcaagagctggatcaacgaggccgacagggacacgatcatcctgaacgcgaagaagatcagcagggagagggacaacggcgagcagtcaacggatacccggagccagaacgtgacggtgagcgttctggacgtgtgcgagaccgctgagaagaagaagctggtgctggtgggcagcggctcaaagaggccagctgctactaagaaggccggccaggctaagaagaagaagtga

SEQ ID NO: 74 - DNA, 2847 bp, synthetic construct
  source 1..2847: mol_type = other DNA
atgggcccaaagaagaagaggaaggtgatggactacaaggaccacgacggcgactacaaggatcacgacatcgactacaaggacgacgacgacaagatgaagaagccgaagcagaacatcgaggagacggacctgaagatcaccaccccaaagaccgcgaccatcaaggccaccaacctggacgacaagatgaggctcttcaccttcttcaacggcttcaccaccgtgtgctccaaggtgaaggacgacatctacaacttcggccagaacgaggacacactgccggtgtacaccgactacattaaggcctcccagagggccaggatgtgcgctactaccctcgctaccaagagcgagtgcgacttcgccaagaagtacggcgagcacttcccgctcccccattacaaccaggagggcatgaactacaccacccaccagcacacctactcagtgaactccgccgtgcacacacagctcgactcccttaacgagtgcgacaagctcaccaacggcgagtacgtcaagctcaagaagaccgtcgacgagctggaggagaagctgaccgaggagcacggcaaggagccacttgatttcctggtgaagttcgtggacgagcagatcctcctgggctggaggttcgacggcaagttcaggctgttcttcgaggtggcgatgctgccagagcttaagaacggcaacatcatctacaagaaggcgtacaagacctccggcggcaagggcaggaggtactctttctacaacccgtccgtggccgataacatttctaagaaccccaccgtgtggaacctgctgagcgacgttaaggcggtggactacatctccctgtctaattccctgctgaggaagaagccgcacgcccagtacaccaacacaaccctgaacagggcccaggtgaggcctacattcggcaacaacggcgtgccattctccatctccgtctccgacgacgactacgtgtacatccgcttcaggctgcccaagaaggacggcgaggagaagggccaggagatctcagtcaagtgcagctacaagacttcatacaagggcaagcgcagcaagacgctgaggaagagctgctacctgggcaacctgaagatcgaggagaatggcaagggcaagtacatttgcaagtacaacatcaacggcagggagacgaccaccgcggagcttaatgagtgcttcctgagggtgaggatcaacaacaaccgctggttcaacaagtacctgaacggcacgctgaccaaggaggacggcgttcttaagagcgagtacttcgacttctacttcgacctgtgcctgaatgtgcatcagaagtccatccacggcctgaccaactccgagattttcggcggcaagggcaagagcatcaggagctactactccacctcctacccggaggtgaagaacctggacggccagaagaacatcaagaccgacttcggctgctacgtggacaagccgcacaacatcatgggcatcgacctgggccagaggaacccattcgcctgggctgttctggaccagaacggcaatgtgaaggacgtgggccacctggacggcgctgagaacgatacatacaaggactacctgacgttctccaacaggtgcaaggacgttaagaatctgatcctgcagtccagggactacctgtacggcgacgatgaggccattgacgagaccctgttcgactccgtggtgcagttcgtgaacagcaacatcacgctgaacaagtacaagtcctacctggacgagaagaagagcctgatcaacaaggagtccctggagaagaaccgcctgtacgagctgaagaagaaggaccacggctggttcgtgagggactgcctttggttcctgaccaaggagtaccacaggatcaactccgagcgcaagacgcactccgactggaggtacaccctgtactgggtggacgccattcaccggttcattgacgtgaacaagtccttcaactccctcggcagctactacgacaagaagcagtccaagtccatcaacggcatccagaaggacttctgcaggagctactggaaccagatcgacaacctgaacgaggacaccctcaagaagttcgtgttcgagctgctgccagtgatcaagaagaacaacgtgtgcctgatcgccatcgaggagctgaagtccatgctgggcgacgacgacaagagggctgaggataacaggctgtacaacctgtggccggtgggccagcttaagacgttcctggagggcaagctgctgccgtacaacgtggctgtgatggaggtgagcgagcagaacacgagccagatcgtgaacggccagtggtcctacagggagggcgatgatctctactacgtgaagaacaacgacaacaacaccatgtgcaagacccacgcggacgagaacgcggctatcaacatcgccctgagggcctactcccaccacactaacctgtactccatctacatgatcaatccgatcgacgactactacgtcccgagctgcatctggaacaacaaggacgagggctccaagaggattaggggcttcctgaccaagacctacggcacctccgacgtggtgttcatcaagaagaatgagaagctggtgaagtccgacgtgagcatcaaggacgtgaagaggatcgtgaagaacatcggcaatgagaagaacaagaagagcgagatctggtacaggatgaacgacatcgagtggatcgacgagggcagcagggacatcatcatcaacacaatcaagagcaaggtgaggggctccggcagcaagaggccagctgctactaagaaggcgggccaggctaagaagaagaagtga

SEQ ID NO: 75 - DNA, 2820 bp, synthetic construct
  source 1..2820: mol_type = other DNA
atgggcccaaagaagaagaggaaggtgatggactacaaggaccacgacggcgactacaaggatcacgacatcgactacaaggacgacgacgacaagatgacggacaagagcatcagcttcaagcagttcagccagatcctcaatgtgctgtacaagtgcatcgtgatttccggcaagggccgcggccttacttccattatcctgggccagccgcagtgcaaggactcacttacctccgccgactggggcaacctggagactctttccgccaaggacgagctgacccctgctgaggttaaggatattaccaaggacctgatgtacagggccagcaacaccctggtctccatcggcttcaggaacaggtcccctttcaagctgaccctgacctccggcgagaggtacgctgttgtggagaacgtgcaccgctccctcaagtcctgggtggaggttgacaagattaccagggagaactacctcaacgaggagatcgccctgagcgatgccttcaataacatcgacgagacgctgctgccaacccttaaggagttcttcgacgcgtgcatgaatgagaacatcatccaccacttcgacgccagggtgtacgcctacacgagggattgcgtcatcccagccctggtggctggccttgagatcaaggaccacttctacatcgacggccgcgacaaggccaagagggattacagcctgcaaggttacgccgagcttctgaagggcttcccgaagctctggcagggcgttgatccggagatcctggctaagctgtacatcctggaggcccagatggaccacaagaagcacaggccatgcgccgcttacgcgttcatcggcgaggattcctacagcagggtgcagtaccttctgggcaacaactacacctccttcagcccctacgccctcggcgttgatctggatgacgtgacctgcggcgatgacgctgaggctgatacacagttccccaagaacaaggtgatccagttcagccagggcaagaaggtgaccaagctgtccctgaccgtgagcaggggcaaggaggataccaacaagtactccttcgatgtgttcctggccgacaagtacagcaacggctcctacaagccaagcccgtacttctctgacctgtccgtttgggtgagcgagatcggcatgctgatggagttcacccgcaagggcgagagggtgcaggctattgtgaaggagccatccctgatttaccgcaagggcgccttctacgtgaggcttaatatgggcgtgattcaggacacctccccggagatcaacgacctgtactggtacttgtcctccggcgccccaatgtccatgaccgataggtccaaggcttccgagaccccgaagaacaccgagaggctggagtcaattaagggcaagagctaccgcttcctgggcatcgacctgggccttaggtccccattcgcctgggctgttggcgaggcttctatctccggcgtcatcaacaagccgacgatcattgccaccggcgactacaccaccgccagggatactaggtacgacacgctcttcttcgccctcaagaatgcgggcaaggtgattggcgtgaccaagtccctcgccaacggcaaggacgcttctttcaatggcctgatgggcaccatcaccgccgctagggagtaccttgcgcactactccggcgtcgctacccataaggtggccgctatccaggccttctgccaggatgacaacccgctggagacccttaagggcctgctcaagtcctacaacaacgacctcgtcaccctcaagaaggaccctaggttcatcggcggcatcctgctcaggtacgccaggcttctgaagggcgagcttgtgacctccaggaagatgcacctgcgggagcactccgtggagtctaagttcggccaggagtacatgtggctgaatattctggagagggagaagagggtgtgcaggagcctgtcctacctgggccttggcaacgacagggacagcgttatcatgggcaacctgaccacgccgtacaaccactgcaaggagaacctgcttaagcagctggccgcgaggattgtgtcactggctgtggagaataagtgccacgttatcgtgatggagtccctgggcggctccaacaagtccatgaataccaggggccagaacttcctcgaggccttctggtccccacagaagatcaaggacaccatcatcaacgccgccgcctggcatggcatcatggttgctgaggtgagcgagagccagacctcccaggtttgcttcgagaccggcaccttcggccacagggatagggcttctctgtacttcctggacaagaacggcgacctccaggagacgcatgccgatatgaacgccgccaagaacctcgtggagaggttcaccaccaggcacaccaacctgaggcaggtgaatatggactccctccccaaggagggcccggataagacaccaaagaagtccccgtccaagaagaagatggagaaggcgaagatggacaacccagaggaccagtccaagaggctcaagggcttcctgaccgtgaagttcggcaatgtgaaggccgcccaggagtacttcgcctctaggaagccggagcagagctacagcggcaagaaggacgaggccatctactggtacttggacggcgacgagtggatcaccaagaaggagaaggagtccagggtcagcgtgattgagggcctggtgggccttaaggaggtggctgttggcagcggctccaagaggccagctgctactaagaaggccggccaggctaagaagaagaagtga

SEQ ID NO: 76 - DNA, 2622 bp, synthetic construct
  source 1..2622: mol_type = other DNA
atgggcccaaagaagaagaggaaggtgatggactacaaggaccacgacggcgactacaaggatcacgacatcgactacaaggacgacgacgacaagatggcgttccagagcaagaggaggattgtgggcaacctggtgaaggagcagtgcctcaaggccgtggatggcaaggtgatcctgaccgaccaggagaagagggagctgatcaagaggtacgagctgcacctggagccgtacaagtggctgctgaggctgttcctgtccggctacgagggcagggatgacggcttctacgaggagctgggcaacacgaacctggacaaggagaagttcttcgaggtcaccgcgggcctcagggatgctcttcttaggcagtctggctcctccagggcgcttaagtcctccatgctgggcaagtgcccgccatcagctgctgttggcaaggctgctaagcacatccaggctctgcgcgacgctggcattcttccattcaagacgggcctcacctccggcgaggattacaacgtgcttcagcaggccgtccagcagctgaggtcatgggttgcttgcgatcacaggaccagggaggcgtacgctgagcagcaggagaagacatcccaggccgaggaggctgctaagaaggctgtgaacgaggtgaagccagaggacgccaagagcctggagaggcatgagagggctctgacgaagctgaggaagcaggagaggaggctggagaggatgaggagccacgctcagttcagcctggacgagatggactgcacgggctacagcctgtgcatgggcgctaactacctgaaggactactgcctggagaaggagggcaggggccttaggcttaccctgaagaatagcactatggccggcagctactacgtttccgtgggcgatggccagcacgctggcatgaagaacccaggtactccggcgggcggctctccagagaagggcaggaggaggaacatcctgttcgacttcgcggttgagaagtgcggcgacaactaccttttcaggtacgacgagaacggcaagcgcccgagggctggcgttgttaaggagccaaggttctgctggaggcggaagggcaactccgtggagctttacctggccatgccgatcaacatcgagaacagcatgaggaacatcttcgtcggcaagcagaagagcggcaagcactccgctttcacccggcagtggccaaaggaggtggagggccttgacgagctgagggatgctgtggtgctgggcgttgacatcggcatcaacagggcggctttctgcgcggctctgaagacttcccgcttcgagaacggcctgccggctgatgttcaggttatggataccacctgcgatgctctgaccgagaagggccaggagtacaggcagctgaggaaggacgccacctgccttgcttggctgatcaggacaaccaggaggttcaaggccgacccaggtaacaagcacaaccagatcaaggagaaggacgtggagaggttcgacagcgccgacggcgcttacaggaggtacatggacgccatcgcggagatgccgtccgatccacttcaggtgtgggaggctgccaggatcaccggctacggcgagtgggctaaggagattttcgccaggttcaatcactacaagcacgagcatgcctgctgcaccgtctccctttccctgtctgaccgcctggtgtggtgcaggcttatcgataggatcttgtctctcaagaagtgccttcacttcggcggctacgagtccaagcacaggaagggcttctgcaagtccctctacaggcttaggcacaatgccaggaacgacgtcaggaagaagctggccaggttcgtggtggacgccgctgttgatgcgggcgcttctgttatcgcgatggaaaagctcccgtcctccggcggcaagcagtctagggatgacaaccggatctgggacctgatggccccaaacaccctggctaccaccgtgtgcctcatggctaaggttgagggcatcggcttcgtgcaggtggacccagagttcacctcccagtgggtgttcgagcagagggtgattggcgatagggagggcaggattgtgtcctgcctggacgctgagggcgtgaggagggattacgacgctgacgagaacgccgcgaagaacatcgcctggctggctcttactagggaggcggagccattctgcatggccttcgagaagcggaatggcgtggtggagccgaagggcttcaggttcgacattccggaggagccgaccagggagcaggatgagtcaaaccaggacttcaagaagaggctggaggagagggacaagctgatcgagaggctgcaggcgaagagcgataggatgagggcgatcgtgaggaggctcttcggcgataggaggccgtgggatgctttcgctgacaggattcctgagggcaagtccaagaggctgttccggcacagggatggcctggttctgaacaagccgttcaagggcctgtgcggctccgagaatagcgagcagaaggcctccgccaggaactctaggggctctggctctaagaggcctgccgctactaagaaggcgggccaggctaagaagaagaagtga

SEQ ID NO: 77 - DNA, 3021 bp, synthetic construct
  source 1..3021: mol_type = other DNA
atgggcccaaagaagaagaggaaggtgatggactacaaggaccacgacggcgactacaaggatcacgacatcgactacaaggacgacgacgacaagatggacacggacacggagctgagcgacgaggttgagctgagcgatgaggtggagctgagcgacgaggtggagctttccgacgaggtggagctgacggtgaagaaggtgaagacgacgacggtgaaggtggacaacaatttcaagaaggagctgttcgagctgttcaatcacttcaccagcgtggcgagcggcatcaaggacaggctttacgacctgcagttcgatgagaacactgcctccatcttcaagggctacatcaaggaggccaagaggggccacggcgctgctactactgtgttcactaagctgaacccgaagaagatctactccggcaagaagtccttcccaagggattacagggaccggggcatcttcccgttctacaacaaggagtctggcaagtacgacctgtccacctgcggctaccactacagcgctaacgccgagattcacacccagctcaacagccacgacgagtgcaacaagcagtgcgagaaggagtacgcggcgctggagaaggagaggaacaagtacaagcatgagttcacgaggcagttcaaggccgagaacgtggagaagttcagcaacttcgtggagaagctgacactgatgggctggaggtacgatgcgaccttcaggaacttcttcgagctgcacatgcacccaaagctcaagacgtccgagaccacctacagggccacctacaagctgccgtccggcaagtctaagcggtactccttctccagggacgatattgccgacgagatcgccaagaaccccgagttctggccaatgctggagtcctccaacgccgtttcctggatcaactccaacaatctgctctccaggaagaaggagaaggccaattactccagcaccagcctgatcaagtcccagattaggctgtacctgggcgacaacggcgtgccattcaccgctagggagcacgatggcaggatctacttcagcttcaggctcccgtccatcaacggcgagaagggcaggaacgtcgagatcccatgctcctacaagaaggtcttcaatggcaaggccaggaagtcctgctacctgggcggccttaccatcgagaacaccggcggctcaaagcacattttcaagtactccgtgaacaacaagaagccgcaggtggcggagctgaacgagtgcttcctgaggctggtcgtgaggaatcatggctacttcaacaagatggtgaacggcaagctcacggataaggacggcaagctgcacgccgactacttcgatttctgcatcgacctgccgcttaacgtgaaggaggacccgatccacgacctgacctaccaggagattaacggcgtgaaggccaacccggagaagaacatcgagaagaaggtgggcctgctgggcttctaccagtccgcttacccagagatcaagaacctcggctcccagatcgagaccggcaagaacctgacctgcccgatcaccaagacccacaacatcatgggcatcgacctcggccagcgcaacccattcgcttactgcatcaaggacaacaacggcaagttcatcgcgaaggaccacatggacggctccaagaacgagacatacaagaagtacatcaatttcggcaaggagagcacctcagtctcccacctgatcaaggagaccaggtcctacctgcatggcgatccggaggctatctccaaggagctgtacaacgaggtcagcggcctgtgcaactctccgcttagctacgaggagtaccttaagtacctggacagcaagaagttcctgatcaacaaggaggacctgaacaagaacgccatgcacctgctgaggcagaaggaccacaactggatcggcagggactggctgtggtacatcagcaagcagtacaagaagcacaacgagaacaggatgcaggacgccgactggaggcagactctgtactggatcgacagcctgtacaggtacatcgatgtgatgaagtccttccacaacttcggcagcttctacgacaagaacctgaagaagaaggtgaacggcaccgccgtgggcttctgcaagactatctacgaccagatcaacaacaacaacaaggacatgttcaagaagttcaccaatgagctgatcccgatcatccgcaagcacaaggtgtccgtggtggcccttgagaagatggagtccatgctgggcgacaagtccaggaacacattcgagaacaggaaccacaacctgtggccagtcggccagctgaagaccttcatcgagaacaagctggatggcttcaacgtgatcgtggtggaggtggacgagaggaacacgagccagatgtgcgacggcaactggtcctacagggaggctgacgacctctactacgtcaaggacggcgagctgagggaggttcacgctgatgagaatgcggccaacaacatcgtcgacaggtgcatctccaggcataccaacatcttcagcctgtacatgaccaacccgatggacgactactacgtgccggcgtgcatctgggacaggtcagagaatggcaagaggggcaggggcttcctgaccaagatgtacaagaacagcgacgtggtgttcaccaagaaggacgacaagctggtgaagtccaagatgtccgtgaaggagctgaagaagctggtggacaagaccaaggagaagaggggccagtactggtacttgttcgagggcaagagctggatcaacgccgccgatagggataccattatctccaacgcgaagaagctcttcagggagagggatggcggcgagcagtcaactgatacccgctctcagaacgtgacggtgtccgtgctggacgtgtgcgagactgtggagaagaagaagctggtcctggtgggctccggctcaaagaggccagctgctactaagaaggccggccaggctaagaagaagaagtga

SEQ ID NO: 78 - DNA, 3162 bp, synthetic construct
  source 1..3162: mol_type = other DNA
atgggcccaaagaagaagaggaaggtgatggactacaaggaccacgacggcgactacaaggatcacgacatcgactacaaggacgacgacgacaagatgagcacggaggtggacgtgaagacgatcaacctgaagatcgcgaagaagggcggcgtgtacccgattctggagcagtcaattaaggagaactgcaagagcaacgacctgctggagttcttcatggtgctgaacaggctgcagacctactacatcgagagcaacgaggagattctggtggacttccccaagaagtacgacgagctgttcgacatcgtgaagaacaacgactcctccgtgaccagggaatacttcgactccctctgcgacaagtacatcacagaggtgtgcgccaatggcttcgtcaacaacgtgtacattgcccacaacaagaaccaggagctgaactgggctgagacgagcaacgaccgcaagatcaagagcaacaagaccttcatgttcggcaagatcaagggcctgatccgcgacaagttcggcagggaggagctgtcagacaaggacgctacgaagcagctgtgcgaggacatcttcaacctcttcatcctgaacaacgccaacatcgagctggacgagaagtacaacatcatcaaggacgagctgatccagatctggaacgagaggaacaaggagttcatccacatcaaggacatcaccctgctgttcaggcagtggggcatcctgcctacctacgacaacatcacccacaactgcgagctgaaggccatcatcgccgagccagtgaggaggttcaagtcctggctggagtgcaactctgaggcgaacaagaactacgacaccgagagggagaagtgcaccaagtacatggacgtgatggactccgacctgaccgtggagttcagcaagatggtgacggagctgggcaacccattcggcgctaacgacaagaacatctacaagtacttcaaccagaagttcctcctgttcttcaagcaggttgtgcagcccaagttcgttaacggcgagccgctggacgagtctaatggctcttactccggcgagatcaagatcaactccgcgggcaaggtggagaactactccatcgccgtgtccgtgattgacaccatcaagaagtacccgacgatctggtccgaccgctcctggggcgagtctgttatctccaccgtggccaagattgatccgcagtacggcatcgacgacatcaccgacgatatgcaggtgtccccgttctacctcttctacggctacttcaccgcctacaactacatccagcagcacaagaggaacgccaagtacaccccgatctccaaggactccctgccatccctgtacctcggcaacaactacatcccattcaagatcgactgcgagaacgtcgacgacgaccggttctacatcaccatcaagaacatgaacaacctgaagctgaacgtcctctaccgcaagcccaagctgaagttcgccaagaccaaggagaagaccaagaggaacaagtgctacttcgacaacctcaagatcaccaacaccaacaacaacttcaagttcgagtacaacatcaacggcgacccaaacaggtccgtggtggcttacctgaaggagccagtgatccgctacaacaacaggaaggactacttctacctgagcgccacaatcagcaaggacgtggagaccgactccgagctgacctctgcttgctggtcgaagatctccaacgacaccgcccgcagggtcaacgctgagcagtacttcaacgacaacggcgtgaacatcgtgggcattgacctgggcatgaacccgatcatcgcctactctgttctgcactacaagaacaacgagttcattgacctgaacattaccggcaagatcgccgacaaggataagcaccccaatctgaactacaagaggatgtacgagaagaggtccgagatcaagaagctcaagaccctgatcaagatgatcccggactacgtgaacagcgacagcaacatcttcgagggcgacaataacgtgttcaagcagctggacaagaagagcaagggcaggttcaggtcctccgagtacatgggctactacgacaagctgaacgtggacggcaagttcatctccgagctggagatcgtgaagaaggtggtgaacacaaagcactacaagaatgacaccgagaagaacaacgatattatgagggtgtacaagggcaataagaagaacatcatcaagaaggagatcgacacccacaggcaccagatccactccatcaaggacatgaacaggaggtccgacgagagcaacctgtgctacgtgtacgacatggtgagctacatcgacgacttcaagaagctggtgacctcctacaacaagatcggcgaggactacaacaacccgatcaagccgctgagcgacccgatgcttttctccaagtccaagctgtacgagtacaggcagaacatcagggacaatttcctgaaggacatctgctaccagatggtgaagatcgccaagcagtacaatgccgtgctggtgcacgagcacttcgagcagaggaagggcggcattgacagggtgaacaacatcctgatggccctgttcacgccgaacgacatcatcaagaagctgaagtgcgtggccaagagggagggcgttctggttttcaacaccaacaagaaccatacctcccagtacgtgtacaacaagaacaccgtcggctaccgcgacagcaacaacaagcacaacctgtactacatcgaggacgagaccaccaggaagctcggcgttgtggactccgacatcaacgcctccaagaacatcgccgcccgcccattcaacaagccactctacgccatcaaggtgaagaactacgatgacggcctgttcctgtcagactacaacaataagtacgttctgtacaagaaggacggcgacaagtacgtggccatcggcgatacatacaggatcgacaagaagaagatcaagcagggctccgtgaccctgtacctgcataacggctactacgtggatggcgagtacaagaacaattacatcgagaatatcaagaagctggtcctgggcagcggcagcaagaggccagctgctactaagaaggccggccaggctaagaagaagaagtga

SEQ ID NO: 79 - DNA, 2622 bp, synthetic construct
  source 1..2622: mol_type = other DNA
atgggcccaaagaagaagaggaaggtgatggactacaaggaccacgacggcgactacaaggatcacgacatcgactacaaggacgacgacgacaagatggcgttccagagcaagaggaggattgtgggcaacttcgtgaaggagcagtgcctgaaggccgtggatggcaaggtgatcctgacggaccaggagaagagggagctgattaagaggtacgagctgcacctggagccgcataagtggctgctgaggctgttcctgtccggctacgagggcagggatgacggcttctacgaggagctgggcaacacgaacctggacaaggagaagttcttcgaggtcaccgcgggcctgagggatgctcttcttaggcagtctggcagcagcagggcgcttaagtcctccatgctgggcaagtgcccgccatcagctgctgttggcaaggctgctaagcacatccagaccctgagggacgccggcattctcccattcaagacgggcctgacctccggcgaggattacaacgtgctgcagcaggccgtgcagcagcttaggtcatgggtggcttgcgaccacaggacgagggaggcttacgctgagcagcaggagaagacaagccaggccgaggaggctgctaagaaggctgctaacgaggtgaagccggaggatgcgaagtctctggagaggcacgagagggtgctgacgaagctgaggaagcaggagaggaggctggagaggatgaagagccacgcgcagttcagcctggacgagatggactgcacgggctactccctgtgcatgggcgctaattacctgaaggactactgcctggagaaggagggcaggggccttaggcttaccctgaagaatagcacgatggctggcagctactacgtttccgtgggcgacggccagcacgctggcatgaagaatccgggcaccccagctggcggctctccagagaagggcaggaggaggaatatcctgttcgacttcaccgtggagaagtgcggcgacaattacctgttcaggtacgacgagaacggcaagaggccgagggctggcgttgttaaggagccaaggttctgctggaggcggaagggcaacagcgtggagctttacctggcgatgccgatcaacatcgagaacagcatgaggaacatcttcgtgggcaagcagaagtccggcaagcactccgctttcacccggcagtggccaaaggaggtcgagggccttgacgagcttagggacgctgtggtgctgggcgttgacatcggcatcaacagggcggctttctgcgccgctctgaagacttccaggttcgagaatggcctgccggccgatgtgcaggttatggataccacctgcgatgcgctgaccgagaagggccaggagtacaggcagctgaggaaggacgccacctgccttgcttggctgatcaggacgaccaggaggttcaaggctgacccaggtaacaagcacaaccagatcaaggagaaggacgtggagaggttcgacagcgccgacggcgcttacaggaggtacatggacgccatcgcggagatgccgagcgatccacttcaggtctgggaggctgccaggatcaccggctacggcgagtgggctaaggagattttcgccaggttcaaccactacaagcatgagcacgcctgctgcgccgtgtctctttctctttccgacaggctggtgtggtgcaggctcatcgacaggatcttgtctctgaagaagtgcctccacttcggcggctacgagtccaagcacaggaagggcttctgcaagtccctgtacaggctgaggcacaacgccaggaacgacgtgaggaagaagctggccaggttcatcgtggatgccgccgttgacgcgggcgcttctgttattgcgatggagaagctgccgtcctctggcggcaagcagtcaaaggacgacaacaggatctgggacctgatggccccgaacaccctggctactactgtgtgcctgatggccaaggtggagggcatcggcttcgtccaggtcgatccagagttcacctcccagtgggtgttcgagcagagggtgattggcgatagggagggcaggatcgtgagctgcctggatgctgagggcgtgaggagggattacgacgctgacgagaacgccgcgaagaacatcgcctggctggctcttaccagggaggctgagccattctgcatggcgttcgagaagaggaacggcgtggtggagccgaagggccttaggttcgacatcccggaggagcctaccagggagcaggatgagtcggaccaggacttcaagaagaggctggaggagagggacaagctgatcgagaggctgcaggcgaaggcggataggatgcaggctatcgttcagaggcttttcggcgacaggaggccgtgggatgctttcgctgacaggattcctgagggcaagagcaagaggctgttcaggcacagggacggcctggttctgaacaagccgttcaagggcctgtgcggctccgagaatagcggccagaaggcttctgctaggaacagccgcggctccggctctaagaggccagctgctactaagaaggcgggccaggctaagaagaagaagtga

SEQ ID NO: 80 - DNA, 35 bp, synthetic construct
  source 1..35: mol_type = other DNA
nnnnnnnnggtataacaacttcgacgagctctaca

SEQ ID NO: 81 - RNA, 27 nt, synthetic construct
  source 1..27: mol_type = other RNA
ggtataacaacttcgacgagctctaca

SEQ ID NO: 82 - RNA, 26 nt, synthetic construct
  source 1..26: mol_type = other RNA
gagccagagaggatcctgggagggag

SEQ ID NO: 83 - RNA, 24 nt, synthetic construct
  source 1..24: mol_type = other RNA
cttccatcagagaacctcactgcg